European Patent Application EP 4 137 572 A1, published February 22, 2023. Title: CHIRAL DESIGN. Applicant: WAVE LIFE SCIENCES PTE. LTD. Application PCT/IB2015/000395. The sequence listing filed with the application follows.

SEQUENCE LISTING (621 sequences)

SEQ ID NO: 1 - DNA, 20 bp, Artificial Sequence
  source: /note="Description of Artificial Sequence: Synthetic oligonucleotide"
gcctcagtctgcttcgcacc

SEQ ID NO: 2 - DNA, 20 bp, Artificial Sequence
  source: /note="Description of Artificial Sequence: Synthetic oligonucleotide"
gcctcagtctgcttcgcacc

SEQ ID NO: 3 - DNA, 13 bp, Artificial Sequence
  source: /note="Description of Artificial Sequence: Synthetic oligonucleotide"
aatcgatcgatcg

SEQ ID NO: 4 - DNA, 20 bp, Artificial Sequence
  source: /note="Description of Artificial Sequence: Synthetic oligonucleotide"
gcctcagtctgcttcgcacc

SEQ ID NO: 5 - DNA, 20 bp, Artificial Sequence
  source: /note="Description of Artificial Sequence: Synthetic oligonucleotide"
gcctcagtctgcttcgcacc

SEQ ID NO: 6 - DNA, 20 bp, Artificial Sequence
  source: /note="Description of Artificial Sequence: Synthetic oligonucleotide"
gcctcagtctgcttcgcacc

SEQ ID NO: 7 - DNA, 20 bp, Artificial Sequence
  source: /note="Description of Artificial Sequence: Synthetic oligonucleotide"
gcctcagtctgcttcgcacc

SEQ ID NO: 8 - RNA, 13 nt, Artificial Sequence
  source: /note="Description of Artificial Sequence: Synthetic oligonucleotide"
gugagcagcugca

SEQ ID NO: 9 - DNA, 20 bp, Artificial Sequence
  source: /note="Description of Artificial Sequence: Synthetic oligonucleotide"
gcctcagtctgcttcgcacc

SEQ ID NO: 10 - DNA, 12 bp, Artificial Sequence
  source: /note="Description of Artificial Sequence: Synthetic oligonucleotide"
cagtctgcttcg

SEQ ID NO: 11 - DNA, 20 bp, Artificial Sequence
  source: /note="Description of Artificial Sequence: Synthetic oligonucleotide"
gcctcagtctgcttcgcacc

SEQ ID NO: 12 - DNA, 12 bp, Artificial Sequence
  source: /note="Description of Artificial Sequence: Synthetic oligonucleotide"
cagtctgcttcg

SEQ ID NO: 13 - DNA, 20 bp, Artificial Sequence
  source: /note="Description of Artificial Sequence: Synthetic oligonucleotide"
gcctcagtctgcttcgcacc

SEQ ID NO: 14 - DNA, 21 bp, Artificial Sequence
  source: /note="Description of Artificial Sequence: Synthetic oligonucleotide"
  source: /note="Description of Combined DNA/RNA Molecule: Synthetic oligonucleotide"
uucuagaccuguuuugcuutt

SEQ ID NO: 15 - DNA, 21 bp, Artificial Sequence
  source: /note="Description of Artificial Sequence: Synthetic oligonucleotide"
  source: /note="Description of Combined DNA/RNA Molecule: Synthetic oligonucleotide"
uucuagaccuguuuugcuutt

SEQ ID NO: 16 - DNA, 21 bp, Artificial Sequence
  source: /note="Description of Artificial Sequence: Synthetic oligonucleotide"
  source: /note="Description of Combined DNA/RNA Molecule: Synthetic oligonucleotide"
aagcaaaacaggucuagaatt

SEQ ID NO: 17 - DNA, 21 bp, Artificial Sequence
  source: /note="Description of Artificial Sequence: Synthetic oligonucleotide"
  source: /note="Description of Combined DNA/RNA Molecule: Synthetic oligonucleotide"
aagcaaaacaggucuagaatt

SEQ ID NO: 18 - DNA, 21 bp, Artificial Sequence
  source: /note="Description of Artificial Sequence: Synthetic oligonucleotide"
  source: /note="Description of Combined DNA/RNA Molecule: Synthetic oligonucleotide"
aagcaaaacaggucuagaatt

SEQ ID NO: 19 - DNA, 20 bp, Artificial Sequence
  source: /note="Description of Artificial Sequence: Synthetic oligonucleotide"
  source: /note="Description of Combined DNA/RNA Molecule: Synthetic oligonucleotide"
agcaaaacaggucuagaatt

SEQ ID NO: 20 - DNA, 20 bp, Artificial Sequence
  source: /note="Description of Artificial Sequence: Synthetic oligonucleotide"
  source: /note="Description of Combined DNA/RNA Molecule: Synthetic oligonucleotide"
agcaaaacaggucuagaatt

SEQ ID NO: 21 - DNA, 20 bp, Artificial Sequence
  source: /note="Description of Artificial Sequence: Synthetic oligonucleotide"
  source: /note="Description of Combined DNA/RNA Molecule: Synthetic oligonucleotide"
agcaaaacaggucuagaatt

SEQ ID NO: 22 - DNA, 21 bp, Artificial Sequence
  source: /note="Description of Artificial Sequence: Synthetic oligonucleotide"
  source: /note="Description of Combined DNA/RNA Molecule: Synthetic oligonucleotide"
uucuagaccuguuuugcuutt

SEQ ID NO: 23 - DNA, 21 bp, Artificial Sequence
  source: /note="Description of Artificial Sequence: Synthetic oligonucleotide"
  source: /note="Description of Combined DNA/RNA Molecule: Synthetic oligonucleotide"
uucuagaccuguuuugcuutt

SEQ ID NO: 24 - DNA, 21 bp, Artificial Sequence
  source: /note="Description of Artificial Sequence: Synthetic oligonucleotide"
  source: /note="Description of Combined DNA/RNA Molecule: Synthetic oligonucleotide"
uucuagaccuguuuugcuutt

SEQ ID NO: 25 - DNA, 21 bp, Artificial Sequence
  source: /note="Description of Artificial Sequence: Synthetic oligonucleotide"
  source: /note="Description of Combined DNA/RNA Molecule: Synthetic oligonucleotide"
uucuagaccuguuuugcuutt

SEQ ID NO: 26 - DNA, 21 bp, Artificial Sequence
  source: /note="Description of Artificial Sequence: Synthetic oligonucleotide"
  source: /note="Description of Combined DNA/RNA Molecule: Synthetic oligonucleotide"
uucuagaccuguuuugcuutt

SEQ ID NO: 27 - DNA, 21 bp, Artificial Sequence
  source: /note="Description of Artificial Sequence: Synthetic oligonucleotide"
  source: /note="Description of Combined DNA/RNA Molecule: Synthetic oligonucleotide"
uucuagaccuguuuugcuutt

SEQ ID NO: 28 - DNA, 21 bp, Artificial Sequence
  source: /note="Description of Artificial Sequence: Synthetic oligonucleotide"
  source: /note="Description of Combined DNA/RNA Molecule: Synthetic oligonucleotide"
aagcaaaacaggucuagaatt

SEQ ID NO: 29 - DNA, 21 bp, Artificial Sequence
  source: /note="Description of Artificial Sequence: Synthetic oligonucleotide"
  source: /note="Description of Combined DNA/RNA Molecule: Synthetic oligonucleotide"
aagcaaaacaggucuagaatt

SEQ ID NO: 30 - DNA, 21 bp, Artificial Sequence
  source: /note="Description of Artificial Sequence: Synthetic oligonucleotide"
  source: /note="Description of Combined DNA/RNA Molecule: Synthetic oligonucleotide"
aagcaaaacaggucuagaatt

SEQ ID NO: 31 - DNA, 21 bp, Artificial Sequence
  source: /note="Description of Artificial Sequence: Synthetic oligonucleotide"
  source: /note="Description of Combined DNA/RNA Molecule: Synthetic oligonucleotide"
aagcaaaacaggucuagaatt

SEQ ID NO: 32 - DNA, 21 bp, Artificial Sequence
  source: /note="Description of Artificial Sequence: Synthetic oligonucleotide"
  source: /note="Description of Combined DNA/RNA Molecule: Synthetic oligonucleotide"
aagcaaaacaggucuagaatt

SEQ ID NO: 33 - DNA, 21 bp, Artificial Sequence
  source: /note="Description of Artificial Sequence: Synthetic oligonucleotide"
  source: /note="Description of Combined DNA/RNA Molecule: Synthetic oligonucleotide"
aagcaaaacaggucuagaatt

SEQ ID NO: 34 - DNA, 21 bp, Artificial Sequence
  source: /note="Description of Artificial Sequence: Synthetic oligonucleotide"
  source: /note="Description of Combined DNA/RNA Molecule: Synthetic oligonucleotide"
aagcaaaacaggucuagaatt

SEQ ID NO: 35 - DNA, 21 bp, Artificial Sequence
  source: /note="Description of Artificial Sequence: Synthetic oligonucleotide"
  source: /note="Description of Combined DNA/RNA Molecule: Synthetic oligonucleotide"
aagcaaaacaggucuagaatt

SEQ ID NO: 36 - DNA, 21 bp, Artificial Sequence
  source: /note="Description of Artificial Sequence: Synthetic oligonucleotide"
  source: /note="Description of Combined DNA/RNA Molecule: Synthetic oligonucleotide"
aagcaaaacaggucuagaatt

SEQ ID NO: 37 - DNA, 21 bp, Artificial Sequence
  source: /note="Description of Artificial Sequence: Synthetic oligonucleotide"
  source: /note="Description of Combined DNA/RNA Molecule: Synthetic oligonucleotide"
aagcaaaacaggucuagaatt

SEQ ID NO: 38 - DNA, 21 bp, Artificial Sequence
  source: /note="Description of Artificial Sequence: Synthetic oligonucleotide"
  source: /note="Description of Combined DNA/RNA Molecule: Synthetic oligonucleotide"
aagcaaaacaggucuagaatt

SEQ ID NO: 39 - DNA, 21 bp, Artificial Sequence
  source: /note="Description of Artificial Sequence: Synthetic oligonucleotide"
  source: /note="Description of Combined DNA/RNA Molecule: Synthetic oligonucleotide"
aagcaaaacaggucuagaatt

SEQ ID NO: 40 - DNA, 21 bp, Artificial Sequence
  source: /note="Description of Artificial Sequence: Synthetic oligonucleotide"
  source: /note="Description of Combined DNA/RNA Molecule: Synthetic oligonucleotide"
uucuagaccuguuuugcuutt

SEQ ID NO: 41 - DNA, 21 bp, Artificial Sequence
  source: /note="Description of Artificial Sequence: Synthetic oligonucleotide"
  source: /note="Description of Combined DNA/RNA Molecule: Synthetic oligonucleotide"
uucuagaccuguuuugcuutt

SEQ ID NO: 42 - DNA, 21 bp, Artificial Sequence
  source: /note="Description of Artificial Sequence: Synthetic oligonucleotide"
  source: /note="Description of Combined DNA/RNA Molecule: Synthetic oligonucleotide"
uucuagaccuguuuugcuutt

SEQ ID NO: 43 - DNA, 21 bp, Artificial Sequence
  source: /note="Description of Artificial Sequence: Synthetic oligonucleotide"
  source: /note="Description of Combined DNA/RNA Molecule: Synthetic oligonucleotide"
uucuagaccuguuuugcuutt

SEQ ID NO: 44 - DNA, 21 bp, Artificial Sequence
  source: /note="Description of Artificial Sequence: Synthetic oligonucleotide"
  source: /note="Description of Combined DNA/RNA Molecule: Synthetic oligonucleotide"
uucuagaccuguuuugcuutt

SEQ ID NO: 45 - DNA, 21 bp, Artificial Sequence
  source: /note="Description of Artificial Sequence: Synthetic oligonucleotide"
  source: /note="Description of Combined DNA/RNA Molecule: Synthetic oligonucleotide"
uucuagaccuguuuugcuutt

SEQ ID NO: 46 - DNA, 21 bp, Artificial Sequence
  source: /note="Description of Artificial Sequence: Synthetic oligonucleotide"
  source: /note="Description of Combined DNA/RNA Molecule: Synthetic oligonucleotide"
aagcaaaacaggucuagaatt

SEQ ID NO: 47 - DNA, 21 bp, Artificial Sequence
  source: /note="Description of Artificial Sequence: Synthetic oligonucleotide"
  source: /note="Description of Combined DNA/RNA Molecule: Synthetic oligonucleotide"
aagcaaaacaggucuagaatt

SEQ ID NO: 48 - DNA, 21 bp, Artificial Sequence
  source: /note="Description of Artificial Sequence: Synthetic oligonucleotide"
  source: /note="Description of Combined DNA/RNA Molecule: Synthetic oligonucleotide"
aagcaaaacaggucuagaatt

SEQ ID NO: 49 - DNA, 21 bp, Artificial Sequence
  source: /note="Description of Artificial Sequence: Synthetic oligonucleotide"
  source: /note="Description of Combined DNA/RNA Molecule: Synthetic oligonucleotide"
aagcaaaacaggucuagaatt

SEQ ID NO: 50 - DNA, 21 bp, Artificial Sequence
  source: /note="Description of Artificial Sequence: Synthetic oligonucleotide"
  source: /note="Description of Combined DNA/RNA Molecule: Synthetic oligonucleotide"
aagcaaaacaggucuagaatt

SEQ ID NO: 51 - DNA, 21 bp, Artificial Sequence
  source: /note="Description of Artificial Sequence: Synthetic oligonucleotide"
  source: /note="Description of Combined DNA/RNA Molecule: Synthetic oligonucleotide"
aagcaaaacaggucuagaatt

SEQ ID NO: 52 - DNA, 21 bp, Artificial Sequence
  source: /note="Description of Artificial Sequence: Synthetic oligonucleotide"
  source: /note="Description of Combined DNA/RNA Molecule: Synthetic oligonucleotide"
aagcaaaacaggucuagaatt

SEQ ID NO: 53 - DNA, 21 bp, Artificial Sequence
  source: /note="Description of Artificial Sequence: Synthetic oligonucleotide"
  source: /note="Description of Combined DNA/RNA Molecule: Synthetic oligonucleotide"
aagcaaaacaggucuagaatt

SEQ ID NO: 54 - DNA, 10 bp, Artificial Sequence
  source: /note="Description of Artificial Sequence: Synthetic oligonucleotide"
acacacacac

SEQ ID NO: 55 - DNA, 10 bp, Artificial Sequence
  source: /note="Description of Artificial Sequence: Synthetic oligonucleotide"
cccccccccc

SEQ ID NO: 56 - DNA, 10 bp, Artificial Sequence
  source: /note="Description of Artificial Sequence: Synthetic oligonucleotide"
cccccccccc

SEQ ID NO: 57 - DNA, 10 bp, Artificial Sequence
  source: /note="Description of Artificial Sequence: Synthetic oligonucleotide"
cccccccccc

SEQ ID NO: 58 - DNA, 12 bp, Artificial Sequence
  source: /note="Description of Artificial Sequence: Synthetic oligonucleotide"
ggatgttctcga

SEQ ID NO: 59 - DNA, 12 bp, Artificial Sequence
  source: /note="Description of Artificial Sequence: Synthetic oligonucleotide"
ggatgttctcga

SEQ ID NO: 60 - DNA, 12 bp, Artificial Sequence
  source: /note="Description of Artificial Sequence: Synthetic oligonucleotide"
ggatgttctcga

SEQ ID NO: 61 - DNA, 16 bp, Artificial Sequence
  source: /note="Description of Artificial Sequence: Synthetic oligonucleotide"
ttcagtcatgacttcc

SEQ ID NO: 62 - DNA, 16 bp, Artificial Sequence
  source: /note="Description of Artificial Sequence: Synthetic oligonucleotide"
ttcagtcatgacttcc

SEQ ID NO: 63 - DNA, 20 bp, Artificial Sequence
  source: /note="Description of Artificial Sequence: Synthetic oligonucleotide"
gcctcagtctgcttcgcacc

SEQ ID NO: 64 - DNA, 20 bp, Artificial Sequence
  source: /note="Description of Artificial Sequence: Synthetic oligonucleotide"
  source: /note="Description of Combined DNA/RNA Molecule: Synthetic oligonucleotide"
  Variation (4)..(4): /replace="u"
  Variation (8)..(8): /replace="u"
  Variation (10)..(10): /replace="u"
  Variation (13)..(14): /replace="u"
  misc_feature (1)..(20): /note="Variant nucleotides given in the sequence have no preference with respect to those in the annotations for variant positions"
gcctcagtctgcttcgcacc

SEQ ID NO: 65 - DNA, 20 bp, Artificial Sequence
  source: /note="Description of Artificial Sequence: Synthetic oligonucleotide"
  source: /note="Description of Combined DNA/RNA Molecule: Synthetic oligonucleotide"
gccucagtctgcttcgcacc

SEQ ID NO: 66 - DNA, 20 bp, Artificial Sequence
  source: /note="Description of Artificial Sequence: Synthetic oligonucleotide"
gcctcagtctgcttcgcacc

SEQ ID NO: 67 - DNA, 20 bp, Artificial Sequence
  source: /note="Description of Artificial Sequence: Synthetic oligonucleotide"
gcctcagtctgcttcgcacc

SEQ ID NO: 68 - DNA, 20 bp, Artificial Sequence
  source: /note="Description of Artificial Sequence: Synthetic oligonucleotide"
gcctcagtctgcttcgcacc

SEQ ID NO: 69 - DNA, 20 bp, Artificial Sequence
  source: /note="Description of Artificial Sequence: Synthetic oligonucleotide"
gcctcagtctgcttcgcacc

SEQ ID NO: 70 - DNA, 20 bp, Artificial Sequence
  source: /note="Description of Artificial Sequence: Synthetic oligonucleotide"
gcctcagtctgcttcgcacc

SEQ ID NO: 71 - DNA, 20 bp, Artificial Sequence
  source: /note="Description of Artificial Sequence: Synthetic oligonucleotide"
gcctcagtctgcttcgcacc

SEQ ID NO: 72 - DNA, 20 bp, Artificial Sequence
  source: /note="Description of Artificial Sequence: Synthetic oligonucleotide"
gcctcagtctgcttcgcacc

SEQ ID NO: 73 - DNA, 20 bp, Artificial Sequence
  source: /note="Description of Artificial Sequence: Synthetic oligonucleotide"
gcctcagtctgcttcgcacc

SEQ ID NO: 74 - DNA, 20 bp, Artificial Sequence
  source: /note="Description of Artificial Sequence: Synthetic oligonucleotide"
gcctcagtctgcttcgcacc

SEQ ID NO: 75 - DNA, 20 bp, Artificial Sequence
  source: /note="Description of Artificial Sequence: Synthetic oligonucleotide"
gcctcagtctgcttcgcacc

SEQ ID NO: 76 - DNA, 20 bp, Artificial Sequence
  source: /note="Description of Artificial Sequence: Synthetic oligonucleotide"
gcctcagtctgcttcgcacc

SEQ ID NO: 77 - DNA, 20 bp, Artificial Sequence
  source: /note="Description of Artificial Sequence: Synthetic oligonucleotide"
gcctcagtctgcttcgcacc

SEQ ID NO: 78 - DNA, 20 bp, Artificial Sequence
  source: /note="Description of Artificial Sequence: Synthetic oligonucleotide"
gcctcagtctgcttcgcacc

SEQ ID NO: 79 - DNA, 20 bp, Artificial Sequence
  source: /note="Description of Artificial Sequence: Synthetic oligonucleotide"
gcctcagtctgcttcgcacc

SEQ ID NO: 80 - DNA, 20 bp, Artificial Sequence
  source: /note="Description of Artificial Sequence: Synthetic oligonucleotide"
gcctcagtctgcttcgcacc

SEQ ID NO: 81 - DNA, 20 bp, Artificial Sequence
  source: /note="Description of Artificial Sequence: Synthetic oligonucleotide"
gcctcagtctgcttcgcacc

SEQ ID NO: 82 - DNA, 20 bp, Artificial Sequence
  source: /note="Description of Artificial Sequence: Synthetic oligonucleotide"
gcctcagtctgcttcgcacc

SEQ ID NO: 83 - DNA, 20 bp, Artificial Sequence
  source: /note="Description of Artificial Sequence: Synthetic oligonucleotide"
gcctcagtctgcttcgcacc

SEQ ID NO: 84 - DNA, 20 bp, Artificial Sequence
  source: /note="Description of Artificial Sequence: Synthetic oligonucleotide"
gcctcagtctgcttcgcacc

SEQ ID NO: 85 - DNA, 20 bp, Artificial Sequence
  source: /note="Description of Artificial Sequence: Synthetic oligonucleotide"
gcctcagtctgcttcgcacc

SEQ ID NO: 86 - DNA, 20 bp, Artificial Sequence
  source: /note="Description of Artificial Sequence: Synthetic oligonucleotide"
gcctcagtctgcttcgcacc

SEQ ID NO: 87 - DNA, 20 bp, Artificial Sequence
  source: /note="Description of Artificial Sequence: Synthetic oligonucleotide"
gcctcagtctgcttcgcacc

SEQ ID NO: 88 - DNA, 20 bp, Artificial Sequence
  source: /note="Description of Artificial Sequence: Synthetic oligonucleotide"
gcctcagtctgcttcgcacc

SEQ ID NO: 89 - DNA, 12 bp, Artificial Sequence
  source: /note="Description of Artificial Sequence: Synthetic oligonucleotide"
cagtctgcttcg

SEQ ID NO: 90 - DNA, 12 bp, Artificial Sequence
  source: /note="Description of Artificial Sequence: Synthetic oligonucleotide"
cagtctgcttcg

SEQ ID NO: 91 - DNA, 12 bp, Artificial Sequence
  source: /note="Description of Artificial Sequence: Synthetic oligonucleotide"
cagtctgcttcg

SEQ ID NO: 92 - DNA, 12 bp, Artificial Sequence
  source: /note="Description of Artificial Sequence: Synthetic oligonucleotide"
cagtctgcttcg

SEQ ID NO: 93 - DNA, 12 bp, Artificial Sequence
  source: /note="Description of Artificial Sequence: Synthetic oligonucleotide"
cagtctgcttcg

SEQ ID NO: 94 - DNA, 12 bp, Artificial Sequence
  source: /note="Description of Artificial Sequence: Synthetic oligonucleotide"
cagtctgcttcg

SEQ ID NO: 95 - DNA, 12 bp, Artificial Sequence
  source: /note="Description of Artificial Sequence: Synthetic oligonucleotide"
cagtctgcttcg

SEQ ID NO: 96 - DNA, 12 bp, Artificial Sequence
  source: /note="Description of Artificial Sequence: Synthetic oligonucleotide"
cagtctgcttcg

SEQ ID NO: 97 - DNA, 12 bp, Artificial Sequence
  source: /note="Description of Artificial Sequence: Synthetic oligonucleotide"
cagtctgcttcg

SEQ ID NO: 98 - DNA, 12 bp, Artificial Sequence
  source: /note="Description of Artificial Sequence: Synthetic oligonucleotide"
cagtctgcttcg

SEQ ID NO: 99 - DNA, 15 bp, Artificial Sequence
  source: /note="Description of Artificial Sequence: Synthetic oligonucleotide"
ctcagtctgcttcgc

SEQ ID NO: 100 - DNA, 12 bp, Artificial Sequence
  source: /note="Description of Artificial Sequence: Synthetic oligonucleotide"
cagtctgcttcg

SEQ ID NO: 101 - DNA, 12 bp, Artificial Sequence
  source: /note="Description of Artificial Sequence: Synthetic oligonucleotide"
cagtctgcttcg

SEQ ID NO: 102 - DNA, 20 bp, Artificial Sequence
  source: /note="Description of Artificial Sequence: Synthetic oligonucleotide"
gcctcagtctgcttcgcacc

SEQ ID NO: 103 - DNA, 20 bp, Artificial Sequence
  source: /note="Description of Artificial Sequence: Synthetic oligonucleotide"
gcctcagtctgcttcgcacc

SEQ ID NO: 104 - DNA, 20 bp, Artificial Sequence
  source: /note="Description of Artificial Sequence: Synthetic oligonucleotide"
gcctcagtctgcttcgcacc

SEQ ID NO: 105 - DNA, 20 bp, Artificial Sequence
  source: /note="Description of Artificial Sequence: Synthetic oligonucleotide"
gcctcagtctgcttcgcacc

SEQ ID NO: 106 - DNA, 20 bp, Artificial Sequence
  source: /note="Description of Artificial Sequence: Synthetic oligonucleotide"
gcctcagtctgcttcgcacc

SEQ ID NO: 107 - DNA, 20 bp, Artificial Sequence
  source: /note="Description of Artificial Sequence: Synthetic oligonucleotide"
gcctcagtctgcttcgcacc

SEQ ID NO: 108 - DNA, 20 bp, Artificial Sequence
  source: /note="Description of Artificial Sequence: Synthetic oligonucleotide"
gcctcagtctgcttcgcacc

SEQ ID NO: 109 - DNA, 20 bp, Artificial Sequence
  source: /note="Description of Artificial Sequence: Synthetic oligonucleotide"
gcctcagtctgcttcgcacc

SEQ ID NO: 110 - DNA, 20 bp, Artificial Sequence
  source: /note="Description of Artificial Sequence: Synthetic oligonucleotide"
gcctcagtctgcttcgcacc

SEQ ID NO: 111 - DNA, 20 bp, Artificial Sequence
  source: /note="Description of Artificial Sequence: Synthetic oligonucleotide"
gcctcagtctgcttcgcacc

SEQ ID NO: 112 - DNA, 20 bp, Artificial Sequence
  source: /note="Description of Artificial Sequence: Synthetic oligonucleotide"
gcctcagtctgcttcgcacc

SEQ ID NO: 113 - DNA, 20 bp, Artificial Sequence
  source: /note="Description of Artificial Sequence: Synthetic oligonucleotide"
gcctcagtctgcttcgcacc

SEQ ID NO: 114 - DNA, 20 bp, Artificial Sequence
  source: /note="Description of Artificial Sequence: Synthetic oligonucleotide"
gcctcagtctgcttcgcacc

SEQ ID NO: 115 - DNA, 20 bp, Artificial Sequence
  source: /note="Description of Artificial Sequence: Synthetic oligonucleotide"
gcctcagtctgcttcgcacc

SEQ ID NO: 116 - DNA, 20 bp, Artificial Sequence
  source: /note="Description of Artificial Sequence: Synthetic oligonucleotide"
gcctcagtctgcttcgcacc

SEQ ID NO: 117 - DNA, 20 bp, Artificial Sequence
  source: /note="Description of Artificial Sequence: Synthetic oligonucleotide"
gcctcagtctgcttcgcacc

SEQ ID NO: 118 - DNA, 20 bp, Artificial Sequence
  source: /note="Description of Artificial Sequence: Synthetic oligonucleotide"
gcctcagtctgcttcgcacc

SEQ ID NO: 119 - DNA, 20 bp, Artificial Sequence
  source: /note="Description of Artificial Sequence: Synthetic oligonucleotide"
gcctcagtctgcttcgcacc

SEQ ID NO: 120 - DNA, 20 bp, Artificial Sequence
  source: /note="Description of Artificial Sequence: Synthetic oligonucleotide"
gcctcagtctgcttcgcacc

SEQ ID NO: 121 - DNA, 20 bp, Artificial Sequence
  source: /note="Description of Artificial Sequence: Synthetic oligonucleotide"
gcctcagtctgcttcgcacc

SEQ ID NO: 122 - DNA, 20 bp, Artificial Sequence
  source: /note="Description of Artificial Sequence: Synthetic oligonucleotide"
gcctcagtctgcttcgcacc

SEQ ID NO: 123 - DNA, 20 bp, Artificial Sequence
  source: /note="Description of Artificial Sequence: Synthetic oligonucleotide"
gcctcagtctgcttcgcacc

SEQ ID NO: 124 - DNA, 20 bp, Artificial Sequence
  source: /note="Description of Artificial Sequence: Synthetic oligonucleotide"
gcctcagtctgcttcgcacc

SEQ ID NO: 125 - DNA, 20 bp, Artificial Sequence
  source: /note="Description of Artificial Sequence: Synthetic oligonucleotide"
gcctcagtctgcttcgcacc

SEQ ID NO: 126 - DNA, 20 bp, Artificial Sequence
  source: /note="Description of Artificial Sequence: Synthetic oligonucleotide"
gcctcagtctgcttcgcacc

SEQ ID NO: 127 - DNA, 20 bp, Artificial Sequence
  source: /note="Description of Artificial Sequence: Synthetic oligonucleotide"
gcctcagtctgcttcgcacc

SEQ ID NO: 128 - DNA, 20 bp, Artificial Sequence
  source: /note="Description of Artificial Sequence: Synthetic oligonucleotide"
gcctcagtctgcttcgcacc

SEQ ID NO: 129 - DNA, 20 bp, Artificial Sequence
  source: /note="Description of Artificial Sequence: Synthetic oligonucleotide"
gcctcagtctgcttcgcacc

SEQ ID NO: 130 - DNA, 20 bp, Artificial Sequence
  source: /note="Description of Artificial Sequence: Synthetic oligonucleotide"
gcctcagtctgcttcgcacc

SEQ ID NO: 131 - DNA, 20 bp, Artificial Sequence
  source: /note="Description of Artificial Sequence: Synthetic oligonucleotide"
  source: /note="Description of Combined DNA/RNA Molecule: Synthetic oligonucleotide"
gcctcagucugcttcgcacc

SEQ ID NO: 132 - DNA, 20 bp, Artificial Sequence
  source: /note="Description of Artificial Sequence: Synthetic oligonucleotide"
gcctcagtctgcttcgcacc

SEQ ID NO: 133 - DNA, 20 bp, Artificial Sequence
  source: /note="Description of Artificial Sequence: Synthetic oligonucleotide"
gcctcagtctgcttcgcacc

SEQ ID NO: 134 - DNA, 20 bp, Artificial Sequence
  source: /note="Description of Artificial Sequence: Synthetic oligonucleotide"
gcctcagtctgcttcgcacc

SEQ ID NO: 135 - DNA, 20 bp, Artificial Sequence
  source: /note="Description of Artificial Sequence: Synthetic oligonucleotide"
gcctcagtctgcttcgcacc

SEQ ID NO: 136 - DNA, 20 bp, Artificial Sequence
  source: /note="Description of Artificial Sequence: Synthetic oligonucleotide"
gcctcagtctgcttcgcacc

SEQ ID NO: 137 - DNA, 20 bp, Artificial Sequence
  source: /note="Description of Artificial Sequence: Synthetic oligonucleotide"
gcctcagtctgcttcgcacc

SEQ ID NO: 138 - DNA, 20 bp, Artificial Sequence
  source: /note="Description of Artificial Sequence: Synthetic oligonucleotide"
gcctcagtctgcttcgcacc

SEQ ID NO: 139 - DNA, 20 bp, Artificial Sequence
  source: /note="Description of Artificial Sequence: Synthetic oligonucleotide"
gcctcagtctgcttcgcacc

SEQ ID NO: 140 - DNA, 20 bp, Artificial Sequence
  source: /note="Description of Artificial Sequence: Synthetic oligonucleotide"
gcctcagtctgcttcgcacc

SEQ ID NO: 141 - DNA, 20 bp, Artificial Sequence
  source: /note="Description of Artificial Sequence: Synthetic oligonucleotide"
gcctcagtctgcttcgcacc

SEQ ID NO: 142 - RNA, 20 nt, Artificial Sequence
  source: /note="Description of Artificial Sequence: Synthetic oligonucleotide"
gccucagucugcuucgcacc

SEQ ID NO: 143 - RNA, 20 nt, Artificial Sequence
  source: /note="Description of Artificial Sequence: Synthetic oligonucleotide"
gccucagucugcuucgcacc

SEQ ID NO: 144 - RNA, 20 nt, Artificial Sequence
  source: /note="Description of Artificial Sequence: Synthetic oligonucleotide"
gccucagucugcuucgcacc

SEQ ID NO: 145 - RNA, 20 nt, Artificial Sequence
  source: /note="Description of Artificial Sequence: Synthetic oligonucleotide"
gccucagucugcuucgcacc

SEQ ID NO: 146 - RNA, 20 nt, Artificial Sequence
  source: /note="Description of Artificial Sequence: Synthetic oligonucleotide"
gccucagucugcuucgcacc

SEQ ID NO: 147 - RNA, 20 nt, Artificial Sequence
  source: /note="Description of Artificial Sequence: Synthetic oligonucleotide"
gccucagucugcuucgcacc

SEQ ID NO: 148 - RNA, 20 nt, Artificial Sequence
  source: /note="Description of Artificial Sequence: Synthetic oligonucleotide"
gccucagucugcuucgcacc

SEQ ID NO: 149 - RNA, 20 nt, Artificial Sequence
  source: /note="Description of Artificial Sequence: Synthetic oligonucleotide"
gccucagucugcuucgcacc

SEQ ID NO: 150 - RNA, 20 nt, Artificial Sequence
  source: /note="Description of Artificial Sequence: Synthetic oligonucleotide"
gccucagucugcuucgcacc

SEQ ID NO: 151 - RNA, 20 nt, Artificial Sequence
  source: /note="Description of Artificial Sequence: Synthetic oligonucleotide"
gccucagucugcuucgcacc

SEQ ID NO: 152 - DNA, 12 bp, Artificial Sequence
  source: /note="Description of Artificial Sequence: Synthetic oligonucleotide"
cagtctgcttcg

SEQ ID NO: 153 - DNA, 20 bp, Artificial Sequence
  source: /note="Description of Artificial Sequence: Synthetic oligonucleotide"
gcctcagtctgcttcgcacc

SEQ ID NO: 154 - DNA, 21 bp, Artificial Sequence
  source: /note="Description of Artificial Sequence: Synthetic oligonucleotide"
  source: /note="Description of Combined DNA/RNA Molecule: Synthetic oligonucleotide"
uucuagaccuguuuugcuutt

SEQ ID NO: 155 - DNA, 21 bp, Artificial Sequence
  source: /note="Description of Artificial Sequence: Synthetic oligonucleotide"
  source: /note="Description of Combined DNA/RNA Molecule: Synthetic oligonucleotide"
uucuagaccuguuuugcuutt

SEQ ID NO: 156 - DNA, 21 bp, Artificial Sequence
  source: /note="Description of Artificial Sequence: Synthetic oligonucleotide"
  source: /note="Description of Combined DNA/RNA Molecule: Synthetic oligonucleotide"
aagcaaaacaggucuagaatt

SEQ ID NO: 157 - DNA, 21 bp, Artificial Sequence
  source: /note="Description of Artificial Sequence: Synthetic oligonucleotide"
  source: /note="Description of Combined DNA/RNA Molecule: Synthetic oligonucleotide"
aagcaaaacaggucuagaatt

SEQ ID NO: 158 - DNA, 21 bp, Artificial Sequence
  source: /note="Description of Artificial Sequence: Synthetic oligonucleotide"
  source: /note="Description of Combined DNA/RNA Molecule: Synthetic oligonucleotide"
aagcaaaacaggucuagaatt

SEQ ID NO: 159 - DNA, 20 bp, Artificial Sequence
  source: /note="Description of Artificial Sequence: Synthetic oligonucleotide"
  source: /note="Description of Combined DNA/RNA Molecule: Synthetic oligonucleotide"
agcaaaacaggucuagaatt

SEQ ID NO: 160 - DNA, 20 bp, Artificial Sequence
  source: /note="Description of Artificial Sequence: Synthetic oligonucleotide"
  source: /note="Description of Combined DNA/RNA Molecule: Synthetic oligonucleotide"
agcaaaacaggucuagaatt

SEQ ID NO: 161 - DNA, 20 bp, Artificial Sequence
  source: /note="Description of Artificial Sequence: Synthetic oligonucleotide"
  source: /note="Description of Combined DNA/RNA Molecule: Synthetic oligonucleotide"
agcaaaacaggucuagaatt

SEQ ID NO: 162 - DNA, 21 bp, Artificial Sequence
  source: /note="Description of Artificial Sequence: Synthetic oligonucleotide"
  source: /note="Description of Combined DNA/RNA Molecule: Synthetic oligonucleotide"
uucuagaccuguuuugcuutt

SEQ ID NO: 163 - DNA, 21 bp, Artificial Sequence
  source: /note="Description of Artificial Sequence: Synthetic oligonucleotide"
  source: /note="Description of Combined DNA/RNA Molecule: Synthetic oligonucleotide"
uucuagaccuguuuugcuutt

SEQ ID NO: 164 - DNA, 21 bp, Artificial Sequence
  source: /note="Description of Artificial Sequence: Synthetic oligonucleotide"
  source: /note="Description of Combined DNA/RNA Molecule: Synthetic oligonucleotide"
uucuagaccuguuuugcuutt

SEQ ID NO: 165 - DNA, 21 bp, Artificial Sequence
  source: /note="Description of Artificial Sequence: Synthetic oligonucleotide"
  source: /note="Description of Combined DNA/RNA Molecule: Synthetic oligonucleotide"
uucuagaccuguuuugcuutt

SEQ ID NO: 166 - DNA, 21 bp, Artificial Sequence
  source: /note="Description of Artificial Sequence: Synthetic oligonucleotide"
  source: /note="Description of Combined DNA/RNA Molecule: Synthetic oligonucleotide"
uucuagaccuguuuugcuutt

SEQ ID NO: 167 - DNA, 21 bp, Artificial Sequence
  source: /note="Description of Artificial Sequence: Synthetic oligonucleotide"
  source: /note="Description of Combined DNA/RNA Molecule: Synthetic oligonucleotide"
uucuagaccuguuuugcuutt

SEQ ID NO: 168 - DNA, 21 bp, Artificial Sequence
  source: /note="Description of Artificial Sequence: Synthetic oligonucleotide"
  source: /note="Description of Combined DNA/RNA Molecule: Synthetic oligonucleotide"
aagcaaaacaggucuagaatt

SEQ ID NO: 169 - DNA, 21 bp, Artificial Sequence
  source: /note="Description of Artificial Sequence: Synthetic oligonucleotide"
  source: /note="Description of Combined DNA/RNA Molecule: Synthetic oligonucleotide"
aagcaaaacaggucuagaatt

SEQ ID NO: 170 - DNA, 21 bp, Artificial Sequence
  source: /note="Description of Artificial Sequence: Synthetic oligonucleotide"
  source: /note="Description of Combined DNA/RNA Molecule: Synthetic oligonucleotide"
aagcaaaacaggucuagaatt

SEQ ID NO: 171 - DNA, 21 bp, Artificial Sequence
  source: /note="Description of Artificial Sequence: Synthetic oligonucleotide"
  source: /note="Description of Combined DNA/RNA Molecule: Synthetic oligonucleotide"
aagcaaaacaggucuagaatt

SEQ ID NO: 172 - DNA, 21 bp, Artificial Sequence
  source: /note="Description of Artificial Sequence: Synthetic oligonucleotide"
  source: /note="Description of Combined DNA/RNA Molecule: Synthetic oligonucleotide"
aagcaaaacaggucuagaatt

SEQ ID NO: 173 - DNA, 21 bp, Artificial Sequence
  source: /note="Description of Artificial Sequence: Synthetic oligonucleotide"
  source: /note="Description of Combined DNA/RNA Molecule: Synthetic oligonucleotide"
aagcaaaacaggucuagaatt

SEQ ID NO: 174 - DNA, 21 bp, Artificial Sequence
  source: /note="Description of Artificial Sequence: Synthetic oligonucleotide"
  source: /note="Description of Combined DNA/RNA Molecule: Synthetic oligonucleotide"
aagcaaaacaggucuagaatt

SEQ ID NO: 175 - DNA, 21 bp, Artificial Sequence
  source: /note="Description of Artificial Sequence: Synthetic oligonucleotide"
  source: /note="Description of Combined DNA/RNA Molecule: Synthetic oligonucleotide"
aagcaaaacaggucuagaatt

SEQ ID NO: 176 - DNA, 21 bp, Artificial Sequence
  source: /note="Description of Artificial Sequence: Synthetic oligonucleotide"
  source: /note="Description of Combined DNA/RNA Molecule: Synthetic oligonucleotide"
aagcaaaacaggucuagaatt

SEQ ID NO: 177 - DNA, 21 bp, Artificial Sequence
  source: /note="Description of Artificial Sequence: Synthetic oligonucleotide"
  source: /note="Description of Combined DNA/RNA Molecule: Synthetic oligonucleotide"
aagcaaaacaggucuagaatt

SEQ ID NO: 178 - DNA, 21 bp, Artificial Sequence
  source: /note="Description of Artificial Sequence: Synthetic oligonucleotide"
  source: /note="Description of Combined DNA/RNA Molecule: Synthetic oligonucleotide"
aagcaaaacaggucuagaatt

SEQ ID NO: 179 - DNA, 21 bp, Artificial Sequence
  source: /note="Description of Artificial Sequence: Synthetic oligonucleotide"
  source: /note="Description of Combined DNA/RNA Molecule: Synthetic oligonucleotide"
aagcaaaacaggucuagaatt

SEQ ID NO: 180 - DNA, 21 bp, Artificial Sequence
  source: /note="Description of Artificial Sequence: Synthetic oligonucleotide"
  source: /note="Description of Combined DNA/RNA Molecule: Synthetic oligonucleotide"
uucuagaccuguuuugcuutt

SEQ ID NO: 181 - DNA, 21 bp, Artificial Sequence
  source: /note="Description of Artificial Sequence: Synthetic oligonucleotide"
  source: /note="Description of Combined DNA/RNA Molecule: Synthetic oligonucleotide"
uucuagaccuguuuugcuutt

SEQ ID NO: 182 - DNA, 21 bp, Artificial Sequence
  source: /note="Description of Artificial Sequence: Synthetic oligonucleotide"
  source: /note="Description of Combined DNA/RNA Molecule: Synthetic oligonucleotide"
uucuagaccuguuuugcuutt

SEQ ID NO: 183 - DNA, 21 bp, Artificial Sequence
  source: /note="Description of Artificial Sequence: Synthetic oligonucleotide"
  source: /note="Description of Combined DNA/RNA Molecule: Synthetic oligonucleotide"
uucuagaccuguuuugcuutt

SEQ ID NO: 184 - DNA, 21 bp, Artificial Sequence
  source: /note="Description of Artificial Sequence: Synthetic oligonucleotide"
  source: /note="Description of Combined DNA/RNA Molecule: Synthetic oligonucleotide"
uucuagaccuguuuugcuutt

SEQ ID NO: 185 - DNA, 21 bp, Artificial Sequence
  source: /note="Description of Artificial Sequence: Synthetic oligonucleotide"
  source: /note="Description of Combined DNA/RNA Molecule: Synthetic oligonucleotide"
uucuagaccuguuuugcuutt

SEQ ID NO: 186 - DNA, 21 bp, Artificial Sequence
  source: /note="Description of Artificial Sequence: Synthetic oligonucleotide"
  source: /note="Description of Combined DNA/RNA Molecule: Synthetic oligonucleotide"
aagcaaaacaggucuagaatt

SEQ ID NO: 187 - DNA, 21 bp, Artificial Sequence
  source: /note="Description of Artificial Sequence: Synthetic oligonucleotide"
  source: /note="Description of Combined DNA/RNA Molecule: Synthetic oligonucleotide"
aagcaaaacaggucuagaatt

SEQ ID NO: 188 - DNA, 21 bp, Artificial Sequence
  source: /note="Description of Artificial Sequence: Synthetic oligonucleotide"
  source: /note="Description of Combined DNA/RNA Molecule: Synthetic oligonucleotide"
aagcaaaacaggucuagaatt

SEQ ID NO: 189 - DNA, 21 bp, Artificial Sequence
  source: /note="Description of Artificial Sequence: Synthetic oligonucleotide"
  source: /note="Description of Combined DNA/RNA Molecule: Synthetic oligonucleotide"
aagcaaaacaggucuagaatt

SEQ ID NO: 190 - DNA, 21 bp, Artificial Sequence
  source: /note="Description of Artificial Sequence: Synthetic oligonucleotide"
  source: /note="Description of Combined DNA/RNA Molecule: Synthetic oligonucleotide"
aagcaaaacaggucuagaatt

SEQ ID NO: 191 - DNA, 21 bp, Artificial Sequence
  source: /note="Description of Artificial Sequence: Synthetic oligonucleotide"
  source: /note="Description of Combined DNA/RNA Molecule: Synthetic oligonucleotide"
aagcaaaacaggucuagaatt

SEQ ID NO: 192 - DNA, 21 bp, Artificial Sequence
  source: /note="Description of Artificial Sequence: Synthetic oligonucleotide"
  source: /note="Description of Combined DNA/RNA Molecule: Synthetic oligonucleotide"
aagcaaaacaggucuagaatt

SEQ ID NO: 193 - DNA, 21 bp, Artificial Sequence
  source: /note="Description of Artificial Sequence: Synthetic oligonucleotide"
  source: /note="Description of Combined DNA/RNA Molecule: Synthetic oligonucleotide"
aagcaaaacaggucuagaatt

SEQ ID NO: 194 - DNA, 12 bp, Artificial Sequence
  source: /note="Description of Artificial Sequence: Synthetic oligonucleotide"
cagtctgcttcg

SEQ ID NO: 195 - DNA, 20 bp, Artificial Sequence
  source: /note="Description of Artificial Sequence: Synthetic oligonucleotide"
gcctcagtctgcttcgcacc

SEQ ID NO: 196 - DNA, 12 bp, Artificial Sequence
  source: /note="Description of Artificial Sequence: Synthetic oligonucleotide"
cagtctgcttcg

SEQ ID NO: 197 - DNA, 20 bp, Artificial Sequence
  source: /note="Description of Artificial Sequence: Synthetic oligonucleotide"
gcctcagtctgcttcgcacc

SEQ ID NO: 198 - DNA, 21 bp, Artificial Sequence
  source: /note="Description of Artificial Sequence: Synthetic oligonucleotide"
  source: /note="Description of Combined DNA/RNA Molecule: Synthetic oligonucleotide"
uucuagaccuguuuugcuutt

SEQ ID NO: 199 - DNA, 21 bp, Artificial Sequence
  source: /note="Description of Artificial Sequence: Synthetic oligonucleotide"
  source: /note="Description of Combined DNA/RNA Molecule: Synthetic oligonucleotide"
uucuagaccuguuuugcuutt

SEQ ID NO: 200 - DNA, 21 bp, Artificial Sequence
  source: /note="Description of Artificial Sequence: Synthetic oligonucleotide"
  source: /note="Description of Combined DNA/RNA Molecule: Synthetic oligonucleotide"
aagcaaaacaggucuagaatt

SEQ ID NO: 201 - DNA, 21 bp, Artificial Sequence
  source: /note="Description of Artificial Sequence: Synthetic oligonucleotide"
  source: /note="Description of Combined DNA/RNA Molecule: Synthetic oligonucleotide"
aagcaaaacaggucuagaatt

SEQ ID NO: 202 - DNA, 21 bp, Artificial Sequence
  source: /note="Description of Artificial Sequence: Synthetic oligonucleotide"
  source: /note="Description of Combined DNA/RNA Molecule: Synthetic oligonucleotide"
aagcaaaacaggucuagaatt

SEQ ID NO: 203 - DNA, 20 bp, Artificial Sequence
  source: /note="Description of Artificial Sequence: Synthetic oligonucleotide"
  source: /note="Description of Combined DNA/RNA Molecule: Synthetic oligonucleotide"
agcaaaacaggucuagaatt

SEQ ID NO: 204 - DNA, 20 bp, Artificial Sequence
  source: /note="Description of Artificial Sequence: Synthetic oligonucleotide"
  source: /note="Description of Combined DNA/RNA Molecule: Synthetic oligonucleotide"
agcaaaacaggucuagaatt

SEQ ID NO: 205 - DNA, 20 bp, Artificial Sequence
  source: /note="Description of Artificial Sequence: Synthetic oligonucleotide"
  source: /note="Description of Combined DNA/RNA Molecule: Synthetic oligonucleotide"
agcaaaacaggucuagaatt

SEQ ID NO: 206 - DNA, 21 bp, Artificial Sequence
  source: /note="Description of Artificial Sequence: Synthetic oligonucleotide"
  source: /note="Description of Combined DNA/RNA Molecule: Synthetic oligonucleotide"
uucuagaccuguuuugcuutt

SEQ ID NO: 207 - DNA, 21 bp, Artificial Sequence
  source: /note="Description of Artificial Sequence: Synthetic oligonucleotide"
  source: /note="Description of Combined DNA/RNA Molecule: Synthetic oligonucleotide"
uucuagaccuguuuugcuutt

SEQ ID NO: 208 - DNA, 21 bp, Artificial Sequence
  source: /note="Description of Artificial Sequence: Synthetic oligonucleotide"
  source: /note="Description of Combined DNA/RNA Molecule: Synthetic oligonucleotide"
uucuagaccuguuuugcuutt

SEQ ID NO: 209 - DNA, 21 bp, Artificial Sequence
  source: /note="Description of Artificial Sequence: Synthetic oligonucleotide"
  source: /note="Description of Combined DNA/RNA Molecule: Synthetic oligonucleotide"
uucuagaccuguuuugcuutt

SEQ ID NO: 210 - DNA, 21 bp, Artificial Sequence
  source: /note="Description of Artificial Sequence: Synthetic oligonucleotide"
  source: /note="Description of Combined DNA/RNA Molecule: Synthetic oligonucleotide"
uucuagaccuguuuugcuutt

SEQ ID NO: 211 - DNA, 21 bp, Artificial Sequence
  source: /note="Description of Artificial Sequence: Synthetic oligonucleotide"
  source: /note="Description of Combined DNA/RNA Molecule: Synthetic oligonucleotide"
uucuagaccuguuuugcuutt

SEQ ID NO: 212 - DNA, 21 bp, Artificial Sequence
  source: /note="Description of Artificial Sequence: Synthetic oligonucleotide"
  source: /note="Description of Combined DNA/RNA Molecule: Synthetic oligonucleotide"
aagcaaaacaggucuagaatt

SEQ ID NO: 213 - DNA, 21 bp, Artificial Sequence
  source: /note="Description of Artificial Sequence: Synthetic oligonucleotide"
  source: /note="Description of Combined DNA/RNA Molecule: Synthetic oligonucleotide"
aagcaaaacaggucuagaatt

SEQ ID NO: 214 - DNA, 21 bp, Artificial Sequence
  source: /note="Description of Artificial Sequence: Synthetic oligonucleotide"
  source: /note="Description of Combined DNA/RNA Molecule: Synthetic oligonucleotide"
aagcaaaacaggucuagaatt

SEQ ID NO: 215 - DNA, 21 bp, Artificial Sequence
  source: /note="Description of Artificial Sequence: Synthetic oligonucleotide"
  source: /note="Description of Combined DNA/RNA Molecule: Synthetic oligonucleotide"
aagcaaaacaggucuagaatt

SEQ ID NO: 216 - DNA, 21 bp, Artificial Sequence
  source: /note="Description of Artificial Sequence: Synthetic oligonucleotide"
  source: /note="Description of Combined DNA/RNA Molecule: Synthetic oligonucleotide"
aagcaaaacaggucuagaatt

SEQ ID NO: 217 - DNA, 21 bp, Artificial Sequence
  source: /note="Description of Artificial Sequence: Synthetic oligonucleotide"
  source: /note="Description of Combined DNA/RNA Molecule: Synthetic oligonucleotide"
aagcaaaacaggucuagaatt

SEQ ID NO: 218 - DNA, 21 bp, Artificial Sequence
  source: /note="Description of Artificial Sequence: Synthetic oligonucleotide"
  source: /note="Description of Combined DNA/RNA Molecule: Synthetic oligonucleotide"
aagcaaaacaggucuagaatt

SEQ ID NO: 219 - DNA, 21 bp, Artificial Sequence
  source: /note="Description of Artificial Sequence: Synthetic oligonucleotide"
  source: /note="Description of Combined DNA/RNA Molecule: Synthetic oligonucleotide"
aagcaaaacaggucuagaatt

SEQ ID NO: 220 - DNA, 21 bp, Artificial Sequence
  source: /note="Description of Artificial Sequence: Synthetic oligonucleotide"
  source: /note="Description of Combined DNA/RNA Molecule: Synthetic oligonucleotide"
aagcaaaacaggucuagaatt

SEQ ID NO: 221 - DNA, 21 bp, Artificial Sequence
  source: /note="Description of Artificial Sequence: Synthetic oligonucleotide"
  source: /note="Description of Combined DNA/RNA Molecule: Synthetic oligonucleotide"
aagcaaaacaggucuagaatt

SEQ ID NO: 222 - DNA, 21 bp, Artificial Sequence
  source: /note="Description of Artificial Sequence: Synthetic oligonucleotide"
  source: /note="Description of Combined DNA/RNA Molecule: Synthetic oligonucleotide"
aagcaaaacaggucuagaatt

SEQ ID NO: 223 - DNA, 21 bp, Artificial Sequence
  source: /note="Description of Artificial Sequence: Synthetic oligonucleotide"
  source: /note="Description of Combined DNA/RNA Molecule: Synthetic oligonucleotide"
aagcaaaacaggucuagaatt

SEQ ID NO: 224 - DNA, 21 bp, Artificial Sequence
  source: /note="Description of Artificial Sequence: Synthetic oligonucleotide"
  source: /note="Description of Combined DNA/RNA Molecule: Synthetic oligonucleotide"
uucuagaccuguuuugcuutt

SEQ ID NO: 225 - DNA, 21 bp, Artificial Sequence
  source: /note="Description of Artificial Sequence: Synthetic oligonucleotide"
  source: /note="Description of Combined DNA/RNA Molecule: Synthetic oligonucleotide"
uucuagaccuguuuugcuutt

SEQ ID NO: 226 - DNA, 21 bp, Artificial Sequence
  source: /note="Description of Artificial Sequence: Synthetic oligonucleotide"
  source: /note="Description of Combined DNA/RNA Molecule: Synthetic oligonucleotide"
uucuagaccuguuuugcuutt

SEQ ID NO: 227 - DNA, 21 bp, Artificial Sequence
  source: /note="Description of Artificial Sequence: Synthetic oligonucleotide"
  source: /note="Description of Combined DNA/RNA Molecule: Synthetic oligonucleotide"
uucuagaccuguuuugcuutt

SEQ ID NO: 228 - DNA, 21 bp, Artificial Sequence
  source: /note="Description of Artificial Sequence: Synthetic oligonucleotide"
  source: /note="Description of Combined DNA/RNA Molecule: Synthetic oligonucleotide"
uucuagaccuguuuugcuutt

SEQ ID NO: 229 - DNA, 21 bp, Artificial Sequence
  source: /note="Description of Artificial Sequence: Synthetic oligonucleotide"
  source: /note="Description of Combined DNA/RNA Molecule: Synthetic oligonucleotide"
uucuagaccuguuuugcuutt

SEQ ID NO: 230 - DNA, 21 bp, Artificial Sequence
  source: /note="Description of Artificial Sequence: Synthetic oligonucleotide"
  source: /note="Description of Combined DNA/RNA Molecule: Synthetic oligonucleotide"
aagcaaaacaggucuagaatt

SEQ ID NO: 231 - DNA, 21 bp, Artificial Sequence
  source: /note="Description of Artificial Sequence: Synthetic oligonucleotide"
  source: /note="Description of Combined DNA/RNA Molecule: Synthetic oligonucleotide"
aagcaaaacaggucuagaatt

SEQ ID NO: 232 - DNA, 21 bp, Artificial Sequence
  source: /note="Description of Artificial Sequence: Synthetic oligonucleotide"
  source: /note="Description of Combined DNA/RNA Molecule: Synthetic oligonucleotide"
aagcaaaacaggucuagaatt

SEQ ID NO: 233 - DNA, 21 bp, Artificial Sequence
  source: /note="Description of Artificial Sequence: Synthetic oligonucleotide"
  source: /note="Description of Combined DNA/RNA Molecule: Synthetic oligonucleotide"
aagcaaaacaggucuagaatt

SEQ ID NO: 234 - DNA, 21 bp, Artificial Sequence
  source: /note="Description of Artificial Sequence: Synthetic oligonucleotide"
  source: /note="Description of Combined DNA/RNA Molecule: Synthetic oligonucleotide"
aagcaaaacaggucuagaatt

SEQ ID NO: 235 - DNA, 21 bp, Artificial Sequence
  source: /note="Description of Artificial Sequence: Synthetic oligonucleotide"
  source: /note="Description of Combined DNA/RNA Molecule: Synthetic oligonucleotide"
aagcaaaacaggucuagaatt

SEQ ID NO: 236 - DNA, 21 bp, Artificial Sequence
  source: /note="Description of Artificial Sequence: Synthetic oligonucleotide"
  source: /note="Description of Combined DNA/RNA Molecule: Synthetic oligonucleotide"
aagcaaaacaggucuagaatt

SEQ ID NO: 237 - DNA, 21 bp, Artificial Sequence
  source: /note="Description of Artificial Sequence: Synthetic oligonucleotide"
  source: /note="Description of Combined DNA/RNA Molecule: Synthetic oligonucleotide"
aagcaaaacaggucuagaatt

SEQ ID NO: 238 - DNA, 27 bp, Artificial Sequence
  source: /note="Description of Artificial Sequence: Synthetic oligonucleotide"
gcgtttgctcttcttcttgcgtttttt

SEQ ID NO: 239 - DNA, 20 bp, Artificial Sequence
  source: /note="Description of Artificial Sequence: Synthetic oligonucleotide"
gcctcagtctgcttcgcacc

SEQ ID NO: 240 - DNA, 20 bp, Artificial Sequence
  source: /note="Description of Artificial Sequence: Synthetic oligonucleotide"
gcctcagtctgcttcgcacc

SEQ ID NO: 241 - DNA, 20 bp, Artificial Sequence
  source: /note="Description of Artificial Sequence: Synthetic oligonucleotide"
gcctcagtctgcttcgcacc

SEQ ID NO: 242 - DNA, 27 bp, Artificial Sequence
  source: /note="Description of Artificial Sequence: Synthetic oligonucleotide"
gcgtttgctcttcttcttgcgtttttt

SEQ ID NO: 243 - DNA, 20 bp, Artificial Sequence
  source: /note="Description of Artificial Sequence: Synthetic oligonucleotide"
gcctcagtctgcttcgcacc

SEQ ID NO: 244 - DNA, 20 bp, Artificial Sequence
  source: /note="Description of Artificial Sequence: Synthetic oligonucleotide"
gcctcagtctgcttcgcacc

SEQ ID NO: 245 - DNA, 20 bp, Artificial Sequence
  source: /note="Description of Artificial Sequence: Synthetic oligonucleotide"
gcctcagtctgcttcgcacc

SEQ ID NO: 246 - DNA, 20 bp, Artificial Sequence
  source: /note="Description of Artificial Sequence: Synthetic oligonucleotide"
gcctcagtctgcttcgcacc

SEQ ID NO: 247 - DNA, 20 bp, Artificial Sequence
  source: /note="Description of Artificial Sequence: Synthetic oligonucleotide"
gcctcagtctgcttcgcacc

SEQ ID NO: 248 - DNA, 20 bp, Artificial Sequence
  source: /note="Description of Artificial Sequence: Synthetic oligonucleotide"
gcctcagtctgcttcgcacc

SEQ ID NO: 249 - DNA, 20 bp, Artificial Sequence
  source: /note="Description of Artificial Sequence: Synthetic oligonucleotide"
gcctcagtctgcttcgcacc

SEQ ID NO: 250 - DNA, 20 bp, Artificial Sequence
  source: /note="Description of Artificial Sequence: Synthetic oligonucleotide"
gcctcagtctgcttcgcacc

SEQ ID NO: 251 - DNA, 27 bp, Artificial Sequence
  source: /note="Description of Artificial Sequence: Synthetic oligonucleotide"
gcgtttgctcttcttcttgcgtttttt

SEQ ID NO: 252 - DNA, 20 bp, Artificial Sequence
  source: /note="Description of Artificial Sequence: Synthetic oligonucleotide"
gtccctgaagatgtcaatgc

SEQ ID NO: 253 - DNA, 20 bp, Artificial Sequence
  source: /note="Description of Artificial Sequence: Synthetic oligonucleotide"
gtccctgaagatgtcaatgc

SEQ ID NO: 254 - DNA, 20 bp, Artificial Sequence
  source: /note="Description of Artificial Sequence: Synthetic oligonucleotide"
gtccctgaagatgtcaatgc

SEQ ID NO: 255 - DNA, 20 bp, Artificial Sequence
  source: /note="Description of Artificial Sequence: Synthetic oligonucleotide"
gtccctgaagatgtcaatgc

SEQ ID NO: 256 - DNA, 20 bp, Artificial Sequence
  source: /note="Description of Artificial Sequence: Synthetic oligonucleotide"
gtccctgaagatgtcaatgc

SEQ ID NO: 257 - DNA, 21 bp, Artificial Sequence
  source: /note="Description of Artificial Sequence: Synthetic oligonucleotide"
  source: /note="Description of Combined DNA/RNA Molecule: Synthetic oligonucleotide"
uucuagaccuguuuugcuutt

SEQ ID NO: 258 - DNA, 21 bp, Artificial Sequence
  source: /note="Description of Artificial Sequence: Synthetic oligonucleotide"
  source: /note="Description of Combined DNA/RNA Molecule: Synthetic oligonucleotide"
uucuagaccuguuuugcuutt

SEQ ID NO: 259 - DNA, 21 bp, Artificial Sequence
  source: /note="Description of Artificial Sequence: Synthetic oligonucleotide"
  source: /note="Description of Combined DNA/RNA Molecule: Synthetic oligonucleotide"
uucuagaccuguuuugcuutt

SEQ ID NO: 260 - DNA, 21 bp, Artificial Sequence
  source: /note="Description of Artificial Sequence: Synthetic oligonucleotide"
  source: /note="Description of Combined DNA/RNA Molecule: Synthetic oligonucleotide"
uucuagaccuguuuugcuutt

SEQ ID NO: 261 - DNA, 21 bp, Artificial Sequence
  source: /note="Description of Artificial Sequence: Synthetic oligonucleotide"
  source: /note="Description of Combined DNA/RNA Molecule: Synthetic oligonucleotide"
uucuagaccuguuuugcuutt

SEQ ID NO: 262 - DNA, 21 bp, Artificial Sequence
  source: /note="Description of Artificial Sequence: Synthetic oligonucleotide"
  source: /note="Description of Combined DNA/RNA Molecule: Synthetic oligonucleotide"
uucuagaccuguuuugcuutt

SEQ ID NO: 263 - DNA, 21 bp, Artificial Sequence
  source: /note="Description of Artificial Sequence: Synthetic oligonucleotide"
  source: /note="Description of Combined DNA/RNA Molecule: Synthetic oligonucleotide"
uucuagaccuguuuugcuutt

SEQ ID NO: 264 - DNA, 21 bp, Artificial Sequence
  source: /note="Description of Artificial Sequence: Synthetic oligonucleotide"
  source: /note="Description of Combined DNA/RNA Molecule: Synthetic oligonucleotide"
uucuagaccuguuuugcuutt

SEQ ID NO: 265 - DNA, 21 bp, Artificial Sequence
  source: /note="Description of Artificial Sequence: Synthetic oligonucleotide"
  source: /note="Description of Combined DNA/RNA Molecule: Synthetic oligonucleotide"
uucuagaccuguuuugcuutt

SEQ ID NO: 266 - DNA, 21 bp, Artificial Sequence
  source: /note="Description of Artificial Sequence: Synthetic oligonucleotide"
  source: /note="Description of Combined DNA/RNA Molecule: Synthetic oligonucleotide"
uucuagaccuguuuugcuutt

SEQ ID NO: 267 - DNA, 21 bp, Artificial Sequence
  source: /note="Description of Artificial Sequence: Synthetic oligonucleotide"
  source: /note="Description of Combined DNA/RNA Molecule: Synthetic oligonucleotide"
uucuagaccuguuuugcuutt

SEQ ID NO: 268 - DNA, 21 bp, Artificial Sequence
  source: /note="Description of Artificial Sequence: Synthetic oligonucleotide"
  source: /note="Description of Combined DNA/RNA Molecule: Synthetic oligonucleotide"
uucuagaccuguuuugcuutt

SEQ ID NO: 269 - DNA, 21 bp, Artificial Sequence
  source: /note="Description of Artificial Sequence: Synthetic oligonucleotide"
  source: /note="Description of Combined DNA/RNA Molecule: Synthetic oligonucleotide"
uucuagaccuguuuugcuutt

SEQ ID NO: 270 - DNA, 21 bp, Artificial Sequence
  source: /note="Description of Artificial Sequence: Synthetic oligonucleotide"
  source: /note="Description of Combined DNA/RNA Molecule: Synthetic oligonucleotide"
uucuagaccuguuuugcuutt

SEQ ID NO: 271 - DNA, 21 bp, Artificial Sequence
  source: /note="Description of Artificial Sequence: Synthetic oligonucleotide"
  source: /note="Description of Combined DNA/RNA Molecule: Synthetic oligonucleotide"
uucuagaccuguuuugcuutt

SEQ ID NO: 272 - DNA, 21 bp, Artificial Sequence
  source: /note="Description of Artificial Sequence: Synthetic oligonucleotide"
  source: /note="Description of Combined DNA/RNA Molecule: Synthetic oligonucleotide"
uucuagaccuguuuugcuutt

SEQ ID NO: 273 - DNA, 21 bp, Artificial Sequence
  source: /note="Description of Artificial Sequence: Synthetic oligonucleotide"
  source: /note="Description of Combined DNA/RNA Molecule: Synthetic oligonucleotide"
uucuagaccuguuuugcuutt

SEQ ID NO: 274 - DNA, 21 bp, Artificial Sequence
  source: /note="Description of Artificial Sequence: Synthetic oligonucleotide"
  source: /note="Description of Combined DNA/RNA Molecule: Synthetic oligonucleotide"
uucuagaccuguuuugcuutt

SEQ ID NO: 275 - DNA, 21 bp, Artificial Sequence
  source: /note="Description of Artificial Sequence: Synthetic oligonucleotide"
  source: /note="Description of Combined DNA/RNA Molecule: Synthetic oligonucleotide"
uucuagaccuguuuugcuutt

SEQ ID NO: 276 - DNA, 21 bp, Artificial Sequence
  source: /note="Description of Artificial Sequence: Synthetic oligonucleotide"
  source: /note="Description of Combined DNA/RNA Molecule: Synthetic oligonucleotide"
uucuagaccuguuuugcuutt

SEQ ID NO: 277 - DNA, 21 bp, Artificial Sequence
  source: /note="Description of Artificial Sequence: Synthetic oligonucleotide"
  source: /note="Description of Combined DNA/RNA Molecule: Synthetic oligonucleotide"
uucuagaccuguuuugcuutt

SEQ ID NO: 278 - DNA, 21 bp, Artificial Sequence
  source: /note="Description of Artificial Sequence: Synthetic oligonucleotide"
  source: /note="Description of Combined DNA/RNA Molecule: Synthetic oligonucleotide"
uucuagaccuguuuugcuutt

SEQ ID NO: 279 - DNA, 21 bp, Artificial Sequence
  source: /note="Description of Artificial Sequence: Synthetic oligonucleotide"
  source: /note="Description of Combined DNA/RNA Molecule: Synthetic oligonucleotide"
uucuagaccuguuuugcuutt

SEQ ID NO: 280 - DNA, 21 bp, Artificial Sequence
  source: /note="Description of Artificial Sequence: Synthetic oligonucleotide"
  source: /note="Description of Combined DNA/RNA Molecule: Synthetic oligonucleotide"
uucuagaccuguuuugcuutt

SEQ ID NO: 281 - DNA, 21 bp, Artificial Sequence
  source: /note="Description of Artificial Sequence: Synthetic oligonucleotide"
  source: /note="Description of Combined DNA/RNA Molecule: Synthetic oligonucleotide"
uucuagaccuguuuugcuutt

SEQ ID NO: 282 - DNA, 21 bp, Artificial Sequence
  source: /note="Description of Artificial Sequence: Synthetic oligonucleotide"
  source: /note="Description of Combined DNA/RNA Molecule: Synthetic oligonucleotide"
uucuagaccuguuuugcuutt

SEQ ID NO: 283 - DNA, 21 bp, Artificial Sequence
  source: /note="Description of Artificial Sequence: Synthetic oligonucleotide"
  source: /note="Description of Combined DNA/RNA Molecule: Synthetic oligonucleotide"
uucuagaccuguuuugcuutt

SEQ ID NO: 284 - DNA, 21 bp, Artificial Sequence
  source: /note="Description of Artificial Sequence: Synthetic oligonucleotide"
  source: /note="Description of Combined DNA/RNA Molecule: Synthetic oligonucleotide"
uucuagaccuguuuugcuutt

SEQ ID NO: 285 - DNA, 21 bp, Artificial Sequence
  source: /note="Description of Artificial Sequence: Synthetic oligonucleotide"
  source: /note="Description of Combined DNA/RNA Molecule: Synthetic oligonucleotide"
uucuagaccuguuuugcuutt

SEQ ID NO: 286 - DNA, 21 bp, Artificial Sequence
  source: /note="Description of Artificial Sequence: Synthetic oligonucleotide"
  source: /note="Description of Combined DNA/RNA Molecule: Synthetic oligonucleotide"
uucuagaccuguuuugcuutt

SEQ ID NO: 287 - DNA, 21 bp, Artificial Sequence
  source: /note="Description of Artificial Sequence: Synthetic oligonucleotide"
  source: /note="Description of Combined DNA/RNA Molecule: Synthetic oligonucleotide"
uucuagaccuguuuugcuutt

SEQ ID NO: 288 - DNA, 21 bp, Artificial Sequence
  source: /note="Description of Artificial Sequence: Synthetic oligonucleotide"
  source: /note="Description of Combined DNA/RNA Molecule: Synthetic oligonucleotide"
uucuagaccuguuuugcuutt

SEQ ID NO: 289 - DNA, 21 bp, Artificial Sequence
  source: /note="Description of Artificial Sequence: Synthetic oligonucleotide"
  source: /note="Description of Combined DNA/RNA Molecule: Synthetic oligonucleotide"
uucuagaccuguuuugcuutt

SEQ ID NO: 290 - DNA, 21 bp, Artificial Sequence
  source: /note="Description of Artificial Sequence: Synthetic oligonucleotide"
  source: /note="Description of Combined DNA/RNA Molecule: Synthetic oligonucleotide"
uucuagaccuguuuugcuutt

SEQ ID NO: 291 - DNA, 21 bp, Artificial Sequence
  source: /note="Description of Artificial Sequence: Synthetic oligonucleotide"
  source: /note="Description of Combined DNA/RNA Molecule: Synthetic oligonucleotide"
uucuagaccuguuuugcuutt

SEQ ID NO: 292 - DNA, 21 bp, Artificial Sequence
  source: /note="Description of Artificial Sequence: Synthetic oligonucleotide"
  source: /note="Description of Combined DNA/RNA Molecule: Synthetic oligonucleotide"
uucuagaccuguuuugcuutt

SEQ ID NO: 293 - DNA, 21 bp, Artificial Sequence
  source: /note="Description of Artificial Sequence: Synthetic oligonucleotide"
  source: /note="Description of Combined DNA/RNA Molecule: Synthetic oligonucleotide"
uucuagaccuguuuugcuutt

SEQ ID NO: 294 - DNA, 21 bp, Artificial Sequence
  source: /note="Description of Artificial Sequence: Synthetic oligonucleotide"
  source: /note="Description of Combined DNA/RNA Molecule: Synthetic oligonucleotide"
uucuagaccuguuuugcuutt

SEQ ID NO: 295 - DNA, 21 bp, Artificial Sequence
  source: /note="Description of Artificial Sequence: Synthetic oligonucleotide"
  source: /note="Description of Combined DNA/RNA Molecule: Synthetic oligonucleotide"
uucuagaccuguuuugcuutt

SEQ ID NO: 296 - DNA, 21 bp, Artificial Sequence
  source: /note="Description of Artificial Sequence: Synthetic oligonucleotide"
  source: /note="Description of Combined DNA/RNA Molecule: Synthetic oligonucleotide"
uucuagaccuguuuugcuutt

SEQ ID NO: 297 - DNA, 21 bp, Artificial Sequence
  source: /note="Description of Artificial Sequence: Synthetic oligonucleotide"
  source: /note="Description of Combined DNA/RNA Molecule: Synthetic oligonucleotide"
aagcaaaacaggucuagaatt

SEQ ID NO: 298 - DNA, 21 bp, Artificial Sequence
  source: /note="Description of Artificial Sequence: Synthetic oligonucleotide"
  source: /note="Description of Combined DNA/RNA Molecule: Synthetic oligonucleotide"
aagcaaaacaggucuagaatt

SEQ ID NO: 299 - DNA, 21 bp, Artificial Sequence
  source: /note="Description of Artificial Sequence: Synthetic oligonucleotide"
  source: /note="Description of Combined DNA/RNA Molecule: Synthetic oligonucleotide"
aagcaaaacaggucuagaatt

SEQ ID NO: 300 - DNA, 21 bp, Artificial Sequence
  source: /note="Description of Artificial Sequence: Synthetic oligonucleotide"
  source: /note="Description of Combined DNA/RNA Molecule: Synthetic oligonucleotide"
aagcaaaacaggucuagaatt

SEQ ID NO: 301 - DNA, 21 bp, Artificial Sequence
  source: /note="Description of Artificial Sequence: Synthetic oligonucleotide"
  source: /note="Description of Combined DNA/RNA Molecule: Synthetic oligonucleotide"
aagcaaaacaggucuagaatt

SEQ ID NO: 302 - DNA, 21 bp, Artificial Sequence
  source: /note="Description of Artificial Sequence: Synthetic oligonucleotide"
  source: /note="Description of Combined DNA/RNA Molecule: Synthetic oligonucleotide"
aagcaaaacaggucuagaatt

SEQ ID NO: 303 - DNA, 21 bp, Artificial Sequence
  source: /note="Description of Artificial Sequence: Synthetic oligonucleotide"
  source: /note="Description of Combined DNA/RNA Molecule: Synthetic oligonucleotide"
aagcaaaacaggucuagaatt

SEQ ID NO: 304 - DNA, 21 bp, Artificial Sequence
  source: /note="Description of Artificial Sequence: Synthetic oligonucleotide"
  source: /note="Description of Combined DNA/RNA Molecule: Synthetic oligonucleotide"
aagcaaaacaggucuagaatt

SEQ ID NO: 305 - DNA, 21 bp, Artificial Sequence
  source: /note="Description of Artificial Sequence: Synthetic oligonucleotide"
  source: /note="Description of Combined DNA/RNA Molecule: Synthetic oligonucleotide"
aagcaaaacaggucuagaatt

SEQ ID NO: 306 - DNA, 21 bp, Artificial Sequence
  source: /note="Description of Artificial Sequence: Synthetic oligonucleotide"
  source: /note="Description of Combined DNA/RNA Molecule: Synthetic oligonucleotide"
aagcaaaacaggucuagaatt

SEQ ID NO: 307 - DNA, 21 bp, Artificial Sequence
  source: /note="Description of Artificial Sequence: Synthetic oligonucleotide"
  source: /note="Description of Combined DNA/RNA Molecule: Synthetic oligonucleotide"
aagcaaaacaggucuagaatt

SEQ ID NO: 308 - DNA, 21 bp, Artificial Sequence
  source: /note="Description of Artificial Sequence: Synthetic oligonucleotide"
  source: /note="Description of Combined DNA/RNA Molecule: Synthetic oligonucleotide"
aagcaaaacaggucuagaatt

SEQ ID NO: 309 - DNA, 21 bp, Artificial Sequence
  source: /note="Description of Artificial Sequence: Synthetic oligonucleotide"
  source: /note="Description of Combined DNA/RNA Molecule: Synthetic oligonucleotide"
aagcaaaacaggucuagaatt

SEQ ID NO: 310 - DNA, 21 bp, Artificial Sequence
  source: /note="Description of Artificial Sequence: Synthetic oligonucleotide"
  source: /note="Description of Combined DNA/RNA Molecule: Synthetic oligonucleotide"
aagcaaaacaggucuagaatt

SEQ ID NO: 311 - DNA, 21 bp, Artificial Sequence
  source: /note="Description of Artificial Sequence: Synthetic oligonucleotide"
  source: /note="Description of Combined DNA/RNA Molecule: Synthetic oligonucleotide"
aagcaaaacaggucuagaatt

SEQ ID NO: 312 - DNA, 21 bp, Artificial Sequence
  source: /note="Description of Artificial Sequence: Synthetic oligonucleotide"
  source: /note="Description of Combined DNA/RNA Molecule: Synthetic oligonucleotide"
aagcaaaacaggucuagaatt

SEQ ID NO: 313 - DNA, 21 bp, Artificial Sequence
  source: /note="Description of Artificial Sequence: Synthetic oligonucleotide"
  source: /note="Description of Combined DNA/RNA Molecule: Synthetic oligonucleotide"
aagcaaaacaggucuagaatt

SEQ ID NO: 314 - DNA, 21 bp, Artificial Sequence
  source: /note="Description of Artificial Sequence: Synthetic oligonucleotide"
  source: /note="Description of Combined DNA/RNA Molecule: Synthetic oligonucleotide"
aagcaaaacaggucuagaatt

SEQ ID NO: 315 - DNA, 21 bp, Artificial Sequence
  source: /note="Description of Artificial Sequence: Synthetic oligonucleotide"
  source: /note="Description of Combined DNA/RNA Molecule: Synthetic oligonucleotide"
aagcaaaacaggucuagaatt

SEQ ID NO: 316 - DNA, 21 bp, Artificial Sequence
  source: /note="Description of Artificial Sequence: Synthetic oligonucleotide"
  source: /note="Description of Combined DNA/RNA Molecule: Synthetic oligonucleotide"
aagcaaaacaggucuagaatt

SEQ ID NO: 317 - DNA, 21 bp, Artificial Sequence
  source: /note="Description of Artificial Sequence: Synthetic oligonucleotide"
  source: /note="Description of Combined DNA/RNA Molecule: Synthetic oligonucleotide"
aagcaaaacaggucuagaatt

SEQ ID NO: 318 - DNA, 21 bp, Artificial Sequence
  source: /note="Description of Artificial Sequence: Synthetic oligonucleotide"
  source: /note="Description of Combined DNA/RNA Molecule: Synthetic oligonucleotide"
aagcaaaacaggucuagaatt

SEQ ID NO: 319 - DNA, 21 bp, Artificial Sequence
  source: /note="Description of Artificial Sequence: Synthetic oligonucleotide"
  source: /note="Description of Combined DNA/RNA Molecule: Synthetic oligonucleotide"
aagcaaaacaggucuagaatt

SEQ ID NO: 320 - DNA, 21 bp, Artificial Sequence
  source: /note="Description of Artificial Sequence: Synthetic oligonucleotide"
  source: /note="Description of Combined DNA/RNA Molecule: Synthetic oligonucleotide"
aagcaaaacaggucuagaatt

SEQ ID NO: 321 - DNA, 21 bp, Artificial Sequence
  source: /note="Description of Artificial Sequence: Synthetic oligonucleotide"
  source: /note="Description of Combined DNA/RNA Molecule: Synthetic oligonucleotide"
aagcaaaacaggucuagaatt

SEQ ID NO: 322 - DNA, 21 bp, Artificial Sequence
  source: /note="Description of Artificial Sequence: Synthetic oligonucleotide"
  source: /note="Description of Combined DNA/RNA Molecule: Synthetic oligonucleotide"
aagcaaaacaggucuagaatt

SEQ ID NO: 323 - DNA, 21 bp, Artificial Sequence
  source: /note="Description of Artificial Sequence: Synthetic oligonucleotide"
  source: /note="Description of Combined DNA/RNA Molecule: Synthetic oligonucleotide"
aagcaaaacaggucuagaatt

SEQ ID NO: 324 - DNA, 21 bp, Artificial Sequence
  source: /note="Description of Artificial Sequence: Synthetic oligonucleotide"
  source: /note="Description of Combined DNA/RNA Molecule: Synthetic oligonucleotide"
aagcaaaacaggucuagaatt

SEQ ID NO: 325 - DNA, 21 bp, Artificial Sequence
  source: /note="Description of Artificial Sequence: Synthetic oligonucleotide"
  source: /note="Description of Combined DNA/RNA Molecule: Synthetic oligonucleotide"
aagcaaaacaggucuagaatt

SEQ ID NO: 326 - DNA, 21 bp, Artificial Sequence
  source: /note="Description of Artificial Sequence: Synthetic oligonucleotide"
  source: /note="Description of Combined DNA/RNA Molecule: Synthetic oligonucleotide"
aagcaaaacaggucuagaatt

SEQ ID NO: 327 - DNA, 21 bp, Artificial Sequence
  source: /note="Description of Artificial Sequence: Synthetic oligonucleotide"
  source: /note="Description of Combined DNA/RNA Molecule: Synthetic oligonucleotide"
aagcaaaacaggucuagaatt

SEQ ID NO: 328 - DNA, 21 bp, Artificial Sequence
  source: /note="Description of Artificial Sequence: Synthetic oligonucleotide"
  source: /note="Description of Combined DNA/RNA Molecule: Synthetic oligonucleotide"
aagcaaaacaggucuagaatt

SEQ ID NO: 329 - DNA, 21 bp, Artificial Sequence
  source: /note="Description of Artificial Sequence: Synthetic oligonucleotide"
  source: /note="Description of Combined DNA/RNA Molecule: Synthetic oligonucleotide"
aagcaaaacaggucuagaatt

SEQ ID NO: 330 - DNA, 21 bp, Artificial Sequence
  source: /note="Description of Artificial Sequence: Synthetic oligonucleotide"
  source: /note="Description of Combined DNA/RNA Molecule: Synthetic oligonucleotide"
aagcaaaacaggucuagaatt

SEQ ID NO: 331 - DNA, 21 bp, Artificial Sequence
  source: /note="Description of Artificial Sequence: Synthetic oligonucleotide"
  source: /note="Description of Combined DNA/RNA Molecule: Synthetic oligonucleotide"
aagcaaaacaggucuagaatt

SEQ ID NO: 332 - DNA, 21 bp, Artificial Sequence
  source: /note="Description of Artificial Sequence: Synthetic oligonucleotide"
  source: /note="Description of Combined DNA/RNA Molecule: Synthetic oligonucleotide"
aagcaaaacaggucuagaatt

SEQ ID NO: 333 - DNA, 21 bp, Artificial Sequence
  source: /note="Description of Artificial Sequence: Synthetic oligonucleotide"
  source: /note="Description of Combined DNA/RNA Molecule: Synthetic oligonucleotide"
aagcaaaacaggucuagaatt

SEQ ID NO: 334 - DNA, 21 bp, Artificial Sequence
  source: /note="Description of Artificial Sequence: Synthetic oligonucleotide"
  source: /note="Description of Combined DNA/RNA Molecule: Synthetic oligonucleotide"
aagcaaaacaggucuagaatt

SEQ ID NO: 335 - DNA, 21 bp, Artificial Sequence
  source: /note="Description of Artificial Sequence: Synthetic oligonucleotide"
  source: /note="Description of Combined DNA/RNA Molecule: Synthetic oligonucleotide"
aagcaaaacaggucuagaatt

SEQ ID NO: 336 - DNA, 21 bp, Artificial Sequence
  source: /note="Description of Artificial Sequence: Synthetic oligonucleotide"
  source: /note="Description of Combined DNA/RNA Molecule: Synthetic oligonucleotide"
aagcaaaacaggucuagaatt

SEQ ID NO: 337 - DNA, 21 bp, Artificial Sequence
  source: /note="Description of Artificial Sequence: Synthetic oligonucleotide"
  source: /note="Description of Combined DNA/RNA Molecule: Synthetic oligonucleotide"
aagcaaaacaggucuagaatt

SEQ ID NO: 338 - DNA, 21 bp, Artificial Sequence
  source: /note="Description of Artificial Sequence: Synthetic oligonucleotide"
  source: /note="Description of Combined DNA/RNA Molecule: Synthetic oligonucleotide"
aagcaaaacaggucuagaatt

SEQ ID NO: 339 - DNA, 21 bp, Artificial Sequence
  source: /note="Description of Artificial Sequence: Synthetic oligonucleotide"
  source: /note="Description of Combined DNA/RNA Molecule: Synthetic oligonucleotide"
aagcaaaacaggucuagaatt

SEQ ID NO: 340 - DNA, 21 bp, Artificial Sequence
  source: /note="Description of Artificial Sequence: Synthetic oligonucleotide"
  source: /note="Description of Combined DNA/RNA Molecule: Synthetic oligonucleotide"
aagcaaaacaggucuagaatt

SEQ ID NO: 341 - DNA, 21 bp, Artificial Sequence
  source: /note="Description of Artificial Sequence: Synthetic oligonucleotide"
  source: /note="Description of Combined DNA/RNA Molecule: Synthetic oligonucleotide"
aagcaaaacaggucuagaatt

SEQ ID NO: 342 - DNA, 21 bp, Artificial Sequence
  source: /note="Description of Artificial Sequence: Synthetic oligonucleotide"
  source: /note="Description of Combined DNA/RNA Molecule: Synthetic oligonucleotide"
aagcaaaacaggucuagaatt

SEQ ID NO: 343 - DNA, 21 bp, Artificial Sequence
  source: /note="Description of Artificial Sequence: Synthetic oligonucleotide"
  source: /note="Description of Combined DNA/RNA Molecule: Synthetic oligonucleotide"
aagcaaaacaggucuagaatt

SEQ ID NO: 344 - DNA, 21 bp, Artificial Sequence
  source: /note="Description of Artificial Sequence: Synthetic oligonucleotide"
  source: /note="Description of Combined DNA/RNA Molecule: Synthetic oligonucleotide"
aagcaaaacaggucuagaatt

SEQ ID NO: 345 - DNA, 21 bp, Artificial Sequence
  source: /note="Description of Artificial Sequence: Synthetic oligonucleotide"
  source: /note="Description of Combined DNA/RNA Molecule: Synthetic oligonucleotide"
aagcaaaacaggucuagaatt

SEQ ID NO: 346 - DNA, 21 bp, Artificial Sequence
  source: /note="Description of Artificial Sequence: Synthetic oligonucleotide"
  source: /note="Description of Combined DNA/RNA Molecule: Synthetic oligonucleotide"
aagcaaaacaggucuagaatt

SEQ ID NO: 347 - DNA, 21 bp, Artificial Sequence
  source: /note="Description of Artificial Sequence: Synthetic oligonucleotide"
  source: /note="Description of Combined DNA/RNA Molecule: Synthetic oligonucleotide"
aagcaaaacaggucuagaatt

SEQ ID NO: 348 - DNA, 21 bp, Artificial Sequence
  source: /note="Description of Artificial Sequence: Synthetic oligonucleotide"
  source: /note="Description of Combined DNA/RNA Molecule: Synthetic oligonucleotide"
aagcaaaacaggucuagaatt

SEQ ID NO: 349 - DNA, 21 bp, Artificial Sequence
  source: /note="Description of Artificial Sequence: Synthetic oligonucleotide"
  source: /note="Description of Combined DNA/RNA Molecule: Synthetic oligonucleotide"
aagcaaaacaggucuagaatt

SEQ ID NO: 350 - DNA, 21 bp, Artificial Sequence
  source: /note="Description of Artificial Sequence: Synthetic oligonucleotide"
  source: /note="Description of Combined DNA/RNA Molecule: Synthetic oligonucleotide"
aagcaaaacaggucuagaatt

SEQ ID NO: 351 - DNA, 21 bp, Artificial Sequence
  source: /note="Description of Artificial Sequence: Synthetic oligonucleotide"
  source: /note="Description of Combined DNA/RNA Molecule: Synthetic oligonucleotide"
aagcaaaacaggucuagaatt

SEQ ID NO: 352 - DNA, 21 bp, Artificial Sequence
  source: /note="Description of Artificial Sequence: Synthetic oligonucleotide"
  source: /note="Description of Combined DNA/RNA Molecule: Synthetic oligonucleotide"
aagcaaaacaggucuagaatt

SEQ ID NO: 353 - DNA, 21 bp, Artificial Sequence
  source: /note="Description of Artificial Sequence: Synthetic oligonucleotide"
  source: /note="Description of Combined DNA/RNA Molecule: Synthetic oligonucleotide"
aagcaaaacaggucuagaatt

SEQ ID NO: 354 - DNA, 21 bp, Artificial Sequence
  source: /note="Description of Artificial Sequence: Synthetic oligonucleotide"
  source: /note="Description of Combined DNA/RNA Molecule: Synthetic oligonucleotide"
aagcaaaacaggucuagaatt

SEQ ID NO: 355 - DNA, 21 bp, Artificial Sequence
  source: /note="Description of Artificial Sequence: Synthetic oligonucleotide"
  source: /note="Description of Combined DNA/RNA Molecule: Synthetic oligonucleotide"
aagcaaaacaggucuagaatt

SEQ ID NO: 356 - DNA, 21 bp, Artificial Sequence
  source: /note="Description of Artificial Sequence: Synthetic oligonucleotide"
  source: /note="Description of Combined DNA/RNA Molecule: Synthetic oligonucleotide"
aagcaaaacaggucuagaatt

SEQ ID NO: 357 - DNA, 21 bp, Artificial Sequence
  source: /note="Description of Artificial Sequence: Synthetic oligonucleotide"
  source: /note="Description of Combined DNA/RNA Molecule: Synthetic oligonucleotide"
aagcaaaacaggucuagaatt

SEQ ID NO: 358 - DNA, 21 bp, Artificial Sequence
  source: /note="Description of Artificial Sequence: Synthetic oligonucleotide"
  source: /note="Description of Combined DNA/RNA Molecule: Synthetic oligonucleotide"
aagcaaaacaggucuagaatt

SEQ ID NO: 359 - DNA, 21 bp, Artificial Sequence
  source: /note="Description of Artificial Sequence: Synthetic oligonucleotide"
  source: /note="Description of Combined DNA/RNA Molecule: Synthetic oligonucleotide"
aagcaaaacaggucuagaatt

SEQ ID NO: 360 - DNA, 21 bp, Artificial Sequence
  source: /note="Description of Artificial Sequence: Synthetic oligonucleotide"
  source: /note="Description of Combined DNA/RNA Molecule: Synthetic oligonucleotide"
aagcaaaacaggucuagaatt

SEQ ID NO: 361 - DNA, 21 bp, Artificial Sequence
  source: /note="Description of Artificial Sequence: Synthetic oligonucleotide"
  source: /note="Description of Combined DNA/RNA Molecule: Synthetic oligonucleotide"
aagcaaaacaggucuagaatt

SEQ ID NO: 362 - DNA, 21 bp, Artificial Sequence
  source: /note="Description of Artificial Sequence: Synthetic oligonucleotide"
  source: /note="Description of Combined DNA/RNA Molecule: Synthetic oligonucleotide"
aagcaaaacaggucuagaatt

SEQ ID NO: 363 - DNA, 21 bp, Artificial Sequence
  source: /note="Description of Artificial Sequence: Synthetic oligonucleotide"
  source: /note="Description of Combined DNA/RNA Molecule: Synthetic oligonucleotide"
aagcaaaacaggucuagaatt

SEQ ID NO: 364 - DNA, 21 bp, Artificial Sequence
  source: /note="Description of Artificial Sequence: Synthetic oligonucleotide"
  source: /note="Description of Combined DNA/RNA Molecule: Synthetic oligonucleotide"
aagcaaaacaggucuagaatt

SEQ ID NO: 365 - DNA, 21 bp, Artificial Sequence
  source: /note="Description of Artificial Sequence: Synthetic oligonucleotide"
  source: /note="Description of Combined DNA/RNA Molecule: Synthetic oligonucleotide"
aagcaaaacaggucuagaatt

SEQ ID NO: 366 - DNA, 21 bp, Artificial Sequence
  source: /note="Description of Artificial Sequence: Synthetic oligonucleotide"
  source: /note="Description of Combined DNA/RNA Molecule: Synthetic oligonucleotide"
aagcaaaacaggucuagaatt

SEQ ID NO: 367 - DNA, 21 bp, Artificial Sequence
  source: /note="Description of Artificial Sequence: Synthetic oligonucleotide"
  source: /note="Description of Combined DNA/RNA Molecule: Synthetic oligonucleotide"
aagcaaaacaggucuagaatt

SEQ ID NO: 368 - DNA, 21 bp, Artificial Sequence
  source: /note="Description of Artificial Sequence: Synthetic oligonucleotide"
  source: /note="Description of Combined DNA/RNA Molecule: Synthetic oligonucleotide"
aagcaaaacaggucuagaatt

SEQ ID NO: 369 - DNA, 21 bp, Artificial Sequence
  source: /note="Description of Artificial Sequence: Synthetic oligonucleotide"
  source: /note="Description of Combined DNA/RNA Molecule: Synthetic oligonucleotide"
aagcaaaacaggucuagaatt

SEQ ID NO: 370 - DNA, 21 bp, Artificial Sequence
  source: /note="Description of Artificial Sequence: Synthetic oligonucleotide"
  source: /note="Description of Combined DNA/RNA Molecule: Synthetic oligonucleotide"
aagcaaaacaggucuagaatt

SEQ ID NO: 371 - DNA, 21 bp, Artificial Sequence
  source: /note="Description of Artificial Sequence: Synthetic oligonucleotide"
  source: /note="Description of Combined DNA/RNA Molecule: Synthetic oligonucleotide"
aagcaaaacaggucuagaatt

SEQ ID NO: 372 - DNA, 21 bp, Artificial Sequence
  source: /note="Description of Artificial Sequence: Synthetic oligonucleotide"
  source: /note="Description of Combined DNA/RNA Molecule: Synthetic oligonucleotide"
aagcaaaacaggucuagaatt

SEQ ID NO: 373 - DNA, 21 bp, Artificial Sequence
  source: /note="Description of Artificial Sequence: Synthetic oligonucleotide"
  source: /note="Description of Combined DNA/RNA Molecule: Synthetic oligonucleotide"
aagcaaaacaggucuagaatt

SEQ ID NO: 374 - DNA, 21 bp, Artificial Sequence
  source: /note="Description of Artificial Sequence: Synthetic oligonucleotide"
  source: /note="Description of Combined DNA/RNA Molecule: Synthetic oligonucleotide"
aagcaaaacaggucuagaatt

SEQ ID NO: 375 - DNA, 21 bp, Artificial Sequence
  source: /note="Description of Artificial Sequence: Synthetic oligonucleotide"
  source: /note="Description of Combined DNA/RNA Molecule: Synthetic oligonucleotide"
aagcaaaacaggucuagaatt

SEQ ID NO: 376 - DNA, 21 bp, Artificial Sequence
  source: /note="Description of Artificial Sequence: Synthetic oligonucleotide"
  source: /note="Description of Combined DNA/RNA Molecule: Synthetic oligonucleotide"
aagcaaaacaggucuagaatt

SEQ ID NO: 377 - DNA, 20 bp, Artificial Sequence
  source: /note="Description of Artificial Sequence: Synthetic oligonucleotide"
ccctctggattgagcatcca

SEQ ID NO: 378 - DNA, 20 bp, Artificial Sequence
  source: /note="Description of Artificial Sequence: Synthetic oligonucleotide"
aagctttggttgggcaacac

SEQ ID NO: 379 - DNA, 20 bp, Artificial Sequence
  source: /note="Description of Artificial Sequence: Synthetic oligonucleotide"
agtcacttgggagcttctcc

SEQ ID NO: 380 - DNA, 20 bp, Artificial Sequence
  source: /note="Description of Artificial Sequence: Synthetic oligonucleotide"
cacttgggagcttctcctgg

SEQ ID NO: 381 - DNA, 20 bp, Artificial Sequence
  source: /note="Description of Artificial Sequence: Synthetic oligonucleotide"
atagccattgcagctgctca

SEQ ID NO: 382 - DNA, 20 bp, Artificial Sequence
  source: /note="Description of Artificial Sequence: Synthetic oligonucleotide"
tggattgagcatccaccaag

SEQ ID NO: 383 - DNA, 20 bp, Artificial Sequence
  source: /note="Description of Artificial Sequence: Synthetic oligonucleotide"
ccatagccattgcagctgct

SEQ ID NO: 384 - DNA, 20 bp, Artificial Sequence
  source: /note="Description of Artificial Sequence: Synthetic oligonucleotide"
gtcacttgggagcttctcct

SEQ ID NO: 385 - DNA, 20 bp, Artificial Sequence
  source: /note="Description of Artificial Sequence: Synthetic oligonucleotide"
ccagggcactcatctgcatg

SEQ ID NO: 386 - DNA, 20 bp, Artificial Sequence
  source: /note="Description of Artificial Sequence: Synthetic oligonucleotide"
gccatccaagtcacttggga

SEQ ID NO: 387 - DNA, 20 bp, Artificial Sequence
  source: /note="Description of Artificial Sequence: Synthetic oligonucleotide"
gaagctttggttgggcaaca

SEQ ID NO: 388 - DNA, 20 bp, Artificial Sequence
  source: /note="Description of Artificial Sequence: Synthetic oligonucleotide"
ctggattgagcatccaccaa

SEQ ID NO: 389 - DNA, 20 bp, Artificial Sequence
  source: /note="Description of Artificial Sequence: Synthetic oligonucleotide"
caagtcacttgggagcttct

SEQ ID NO: 390 - DNA, 20 bp, Artificial Sequence
  source: /note="Description of Artificial Sequence: Synthetic oligonucleotide"
atgccatccaagtcacttgg

SEQ ID NO: 391 - DNA, 20 bp, Artificial Sequence
  source: /note="Description of Artificial Sequence: Synthetic oligonucleotide"
atgagatgcctggctgccat

SEQ ID NO: 392 - DNA, 20 bp, Artificial Sequence
  source: /note="Description of Artificial Sequence: Synthetic oligonucleotide"
ttgggagcttctcctggtgg

SEQ ID NO: 393 - DNA, 20 bp, Artificial Sequence
  source: /note="Description of Artificial Sequence: Synthetic oligonucleotide"
tgggagcttctcctggtgga

SEQ ID NO: 394 - DNA, 20 bp, Artificial Sequence
  source: /note="Description of Artificial Sequence: Synthetic oligonucleotide"
ttatgagatgcctggctgcc

SEQ ID NO: 395 - DNA, 20 bp, Artificial Sequence
  source: /note="Description of Artificial Sequence: Synthetic oligonucleotide"
gttatgagatgcctggctgc

SEQ ID NO: 396 - DNA, 20 bp, Artificial Sequence
  source: /note="Description of Artificial Sequence: Synthetic oligonucleotide"
ccaagtcacttgggagcttc

SEQ ID NO: 397 - DNA, 20 bp, Artificial Sequence
  source: /note="Description of Artificial Sequence: Synthetic oligonucleotide"
agctttggttgggcaacaca

SEQ ID NO: 398 - DNA, 20 bp, Artificial Sequence
  source: /note="Description of Artificial Sequence: Synthetic oligonucleotide"
tatgagatgcctggctgcca

SEQ ID NO: 399 - DNA, 20 bp, Artificial Sequence
  source: /note="Description of Artificial Sequence: Synthetic oligonucleotide"
tgttatgagatgcctggctg

SEQ ID NO: 400 - DNA, 20 bp, Artificial Sequence
  source: /note="Description of Artificial Sequence: Synthetic oligonucleotide"
atccaagtcacttgggagct

SEQ ID NO: 401 - DNA, 20 bp, Artificial Sequence
  source: /note="Description of Artificial Sequence: Synthetic oligonucleotide"
gggaagctttggttgggcaa

SEQ ID NO: 402 - DNA, 20 bp, Artificial Sequence
  source: /note="Description of Artificial Sequence: Synthetic oligonucleotide"
ctccatccatgaggtcattc

SEQ ID NO: 403 - DNA, 20 bp, Artificial Sequence
  source: /note="Description of Artificial Sequence: Synthetic oligonucleotide"
aagtcacttgggagcttctc

SEQ ID NO: 404 - DNA, 20 bp, Artificial Sequence
  source: /note="Description of Artificial Sequence: Synthetic oligonucleotide"
ccatccaagtcacttgggag

SEQ ID NO: 405 - DNA, 20 bp, Artificial Sequence
  source: /note="Description of Artificial Sequence: Synthetic oligonucleotide"
tccaagtcacttgggagctt

SEQ ID NO: 406 - DNA, 20 bp, Artificial Sequence
  source: /note="Description of Artificial Sequence: Synthetic oligonucleotide"
cctctggattgagcatccac

SEQ ID NO: 407 - DNA, 20 bp, Artificial Sequence
  source: /note="Description of Artificial Sequence: Synthetic oligonucleotide"
acttgggagcttctcctggt

SEQ ID NO: 408 - DNA, 20 bp, Artificial Sequence
  source: /note="Description of Artificial Sequence: Synthetic oligonucleotide"
cttgggagcttctcctggtg

SEQ ID NO: 409 - DNA, 20 bp, Artificial Sequence
  source: /note="Description of Artificial Sequence: Synthetic oligonucleotide"
catgccatccaagtcacttg

SEQ ID NO: 410 - DNA, 20 bp, Artificial Sequence
  source: /note="Description of Artificial Sequence: Synthetic oligonucleotide"
tgccatccaagtcacttggg

SEQ ID NO: 411 - DNA, 20 bp, Artificial Sequence
  source: /note="Description of Artificial Sequence: Synthetic oligonucleotide"
tccatccatgaggtcattcc

SEQ ID NO: 412 - DNA, 20 bp, Artificial Sequence
  source: /note="Description of Artificial Sequence: Synthetic oligonucleotide"
agggcactcatctgcatggg

SEQ ID NO: 413 - DNA, 20 bp, Artificial Sequence
  source: /note="Description of Artificial Sequence: Synthetic oligonucleotide"
ccagttccttcattctgcac

SEQ ID NO: 414 - DNA, 20 bp, Artificial Sequence
  source: /note="Description of Artificial Sequence: Synthetic oligonucleotide"
catagccattgcagctgctc

SEQ ID NO: 415 - DNA, 20 bp, Artificial Sequence
  source: /note="Description of Artificial Sequence: Synthetic oligonucleotide"
tctggattgagcatccacca

SEQ ID NO: 416 - DNA, 20 bp, Artificial Sequence
  source: /note="Description of Artificial Sequence: Synthetic oligonucleotide"
ggattgagcatccaccaaga

SEQ ID NO: 417 - DNA, 20 bp, Artificial Sequence
  source: /note="Description of Artificial Sequence: Synthetic oligonucleotide"
ccctctggattgagcatcca

SEQ ID NO: 418 - DNA, 20 bp, Artificial Sequence
  source: /note="Description of Artificial Sequence: Synthetic oligonucleotide"
aagctttggttgggcaacac

SEQ ID NO: 419 - DNA, 20 bp, Artificial Sequence
  source: /note="Description of Artificial Sequence: Synthetic oligonucleotide"
agtcacttgggagcttctcc

SEQ ID NO: 420 - DNA, 20 bp, Artificial Sequence
  source: /note="Description of Artificial Sequence: Synthetic oligonucleotide"
cacttgggagcttctcctgg

SEQ ID NO: 421 - DNA, 20 bp, Artificial Sequence
  source: /note="Description of Artificial Sequence: Synthetic oligonucleotide"
atagccattgcagctgctca

SEQ ID NO: 422 - DNA, 20 bp, Artificial Sequence
  source: /note="Description of Artificial Sequence: Synthetic oligonucleotide"
tggattgagcatccaccaag

SEQ ID NO: 423 - DNA, 20 bp, Artificial Sequence
  source: /note="Description of Artificial Sequence: Synthetic oligonucleotide"
ccatagccattgcagctgct

SEQ ID NO: 424 - DNA, 20 bp, Artificial Sequence
  source: /note="Description of Artificial Sequence: Synthetic oligonucleotide"
gtcacttgggagcttctcct

SEQ ID NO: 425 - DNA, 20 bp, Artificial Sequence
  source: /note="Description of Artificial Sequence: Synthetic oligonucleotide"
ccagggcactcatctgcatg

SEQ ID NO: 426 - DNA, 20 bp, Artificial Sequence
  source: /note="Description of Artificial Sequence: Synthetic oligonucleotide"
gccatccaagtcacttggga

SEQ ID NO: 427 - DNA, 20 bp, Artificial Sequence
  source: /note="Description of Artificial Sequence: Synthetic oligonucleotide"
gaagctttggttgggcaaca

SEQ ID NO: 428 - DNA, 20 bp, Artificial Sequence
  source: /note="Description of Artificial Sequence: Synthetic oligonucleotide"
ctggattgagcatccaccaa

SEQ ID NO: 429 - DNA, 20 bp, Artificial Sequence
  source: /note="Description of Artificial Sequence: Synthetic oligonucleotide"
caagtcacttgggagcttct

SEQ ID NO: 430 - DNA, 20 bp, Artificial Sequence
  source: /note="Description of Artificial Sequence: Synthetic oligonucleotide"
atgccatccaagtcacttgg

SEQ ID NO: 431 - DNA, 20 bp, Artificial Sequence
  source: /note="Description of Artificial Sequence: Synthetic oligonucleotide"
atgagatgcctggctgccat

SEQ ID NO: 432 - DNA, 20 bp, Artificial Sequence
  source: /note="Description of Artificial Sequence: Synthetic oligonucleotide"
ttgggagcttctcctggtgg

SEQ ID NO: 433 - DNA, 20 bp, Artificial Sequence
  source: /note="Description of Artificial Sequence: Synthetic oligonucleotide"
tgggagcttctcctggtgga

SEQ ID NO: 434 - DNA, 20 bp, Artificial Sequence
  source: /note="Description of Artificial Sequence: Synthetic oligonucleotide"
ttatgagatgcctggctgcc

SEQ ID NO: 435 - DNA, 20 bp, Artificial Sequence
  source: /note="Description of Artificial Sequence: Synthetic oligonucleotide"
gttatgagatgcctggctgc

SEQ ID NO: 436 - DNA, 20 bp, Artificial Sequence
  source: /note="Description of Artificial Sequence: Synthetic oligonucleotide"
ccaagtcacttgggagcttc

SEQ ID NO: 437 - DNA, 20 bp, Artificial Sequence
  source: /note="Description of Artificial Sequence: Synthetic oligonucleotide"
agctttggttgggcaacaca

SEQ ID NO: 438 - DNA, 20 bp, Artificial Sequence
  source: /note="Description of Artificial Sequence: Synthetic oligonucleotide"
tatgagatgcctggctgcca

SEQ ID NO: 439 - DNA, 20 bp, Artificial Sequence
  source: /note="Description of Artificial Sequence: Synthetic oligonucleotide"
tgttatgagatgcctggctg

SEQ ID NO: 440 - DNA, 20 bp, Artificial Sequence
  source: /note="Description of Artificial Sequence: Synthetic oligonucleotide"
atccaagtcacttgggagct

SEQ ID NO: 441 - DNA, 20 bp, Artificial Sequence
  source: /note="Description of Artificial Sequence: Synthetic oligonucleotide"
gggaagctttggttgggcaa

SEQ ID NO: 442 - DNA, 20 bp, Artificial Sequence
  source: /note="Description of Artificial Sequence: Synthetic oligonucleotide"
ctccatccatgaggtcattc

SEQ ID NO: 443 - DNA, 20 bp, Artificial Sequence
  source: /note="Description of Artificial Sequence: Synthetic oligonucleotide"
aagtcacttgggagcttctc

SEQ ID NO: 444 - DNA, 20 bp, Artificial Sequence
  source: /note="Description of Artificial Sequence: Synthetic oligonucleotide"
ccatccaagtcacttgggag

SEQ ID NO: 445 - DNA, 20 bp, Artificial Sequence
  source: /note="Description of Artificial Sequence: Synthetic oligonucleotide"
tccaagtcacttgggagctt

SEQ ID NO: 446 - DNA, 20 bp, Artificial Sequence
  source: /note="Description of Artificial Sequence: Synthetic oligonucleotide"
cctctggattgagcatccac

SEQ ID NO: 447 - DNA, 20 bp, Artificial Sequence
  source: /note="Description of Artificial Sequence: Synthetic oligonucleotide"
acttgggagcttctcctggt

SEQ ID NO: 448 - DNA, 20 bp, Artificial Sequence
  source: /note="Description of Artificial Sequence: Synthetic oligonucleotide"
cttgggagcttctcctggtg

SEQ ID NO: 449 - DNA, 20 bp, Artificial Sequence
  source: /note="Description of Artificial Sequence: Synthetic oligonucleotide"
catgccatccaagtcacttg

SEQ ID NO: 450 - DNA, 20 bp, Artificial Sequence
  source: /note="Description of Artificial Sequence: Synthetic oligonucleotide"
tgccatccaagtcacttggg

SEQ ID NO: 451 - DNA, 20 bp, Artificial Sequence
  source: /note="Description of Artificial Sequence: Synthetic oligonucleotide"
tccatccatgaggtcattcc

SEQ ID NO: 452 - DNA, 20 bp, Artificial Sequence
  source: /note="Description of Artificial Sequence: Synthetic oligonucleotide"
agggcactcatctgcatggg

SEQ ID NO: 453 - DNA, 20 bp, Artificial Sequence
  source: /note="Description of Artificial Sequence: Synthetic oligonucleotide"
ccagttccttcattctgcac

SEQ ID NO: 454 - DNA, 20 bp, Artificial Sequence
  source: /note="Description of Artificial Sequence: Synthetic oligonucleotide"
catagccattgcagctgctc

SEQ ID NO: 455 - DNA, 20 bp, Artificial Sequence
  source: /note="Description of Artificial Sequence: Synthetic oligonucleotide"
tctggattgagcatccacca

SEQ ID NO: 456 - DNA, 20 bp, Artificial Sequence
  source: /note="Description of Artificial Sequence: Synthetic oligonucleotide"
ggattgagcatccaccaaga

SEQ ID NO: 457 - DNA, 20 bp, Artificial Sequence
  source: /note="Description of Artificial Sequence: Synthetic oligonucleotide"
gaagctttggttgggcaaca

SEQ ID NO: 458 - DNA, 20 bp, Artificial Sequence
  source: /note="Description of Artificial Sequence: Synthetic oligonucleotide"
ccatccaagtcacttgggag

SEQ ID NO: 459 - DNA, 20 bp, Artificial Sequence
  source: /note="Description of Artificial Sequence: Synthetic oligonucleotide"
atgagatgcctggctgccat

SEQ ID NO: 460 - DNA, 20 bp, Artificial Sequence
  source: /note="Description of Artificial Sequence: Synthetic oligonucleotide"
aagctttggttgggcaacac

SEQ ID NO: 461 - DNA, 20 bp, Artificial Sequence
  source: /note="Description of Artificial Sequence: Synthetic oligonucleotide"
atagccattgcagctgctca

SEQ ID NO: 462 - DNA, 20 bp, Artificial Sequence
  source: /note="Description of Artificial Sequence: Synthetic oligonucleotide"
tatgagatgcctggctgcca

SEQ ID NO: 463 - DNA, 20 bp, Artificial Sequence
  source: /note="Description of Artificial Sequence: Synthetic oligonucleotide"
ttatgagatgcctggctgcc

SEQ ID NO: 464 - DNA, 20 bp, Artificial Sequence
  source: /note="Description of Artificial Sequence: Synthetic oligonucleotide"
ccatccaagtcacttgggag

SEQ ID NO: 465 - DNA, 20 bp, Artificial Sequence
  source: /note="Description of Artificial Sequence: Synthetic oligonucleotide"
ccatccaagtcacttgggag

SEQ ID NO: 466 - DNA, 20 bp, Artificial Sequence
  source: /note="Description of Artificial Sequence: Synthetic oligonucleotide"
gaagctttggttgggcaaca

SEQ ID NO: 467 - DNA, 20 bp, Artificial Sequence
  source: /note="Description of Artificial Sequence: Synthetic oligonucleotide"
ccatccaagtcacttgggag

SEQ ID NO: 468 - DNA, 20 bp, Artificial Sequence
  source: /note="Description of Artificial Sequence: Synthetic oligonucleotide"
ccatccaagtcacttgggag

SEQ ID NO: 469 - DNA, 20 bp, Artificial Sequence
  source: /note="Description of Artificial Sequence: Synthetic oligonucleotide"
gaagctttggttgggcaaca

SEQ ID NO: 470 - DNA, 20 bp, Artificial Sequence
  source: /note="Description of Artificial Sequence: Synthetic oligonucleotide"
atgagatgcctggctgccat

SEQ ID NO: 471 - DNA, 20 bp, Artificial Sequence
  source: /note="Description of Artificial Sequence: Synthetic oligonucleotide"
atgagatgcctggctgccat

SEQ ID NO: 472 - DNA, 20 bp, Artificial Sequence
  source: /note="Description of Artificial Sequence: Synthetic oligonucleotide"
atgagatgcctggctgccat

SEQ ID NO: 473 - DNA, 20 bp, Artificial Sequence
  source: /note="Description of Artificial Sequence: Synthetic oligonucleotide"
atgagatgcctggctgccat

SEQ ID NO: 474 - DNA, 20 bp, Artificial Sequence
  source: /note="Description of Artificial Sequence: Synthetic oligonucleotide"
gaagctttggttgggcaaca

SEQ ID NO: 475 - DNA, 20 bp, Artificial Sequence
  source: /note="Description of Artificial Sequence: Synthetic oligonucleotide"
ccatccaagtcacttgggag

SEQ ID NO: 476 - DNA, 20 bp, Artificial Sequence
  source: /note="Description of Artificial Sequence: Synthetic oligonucleotide"
atgagatgcctggctgccat

SEQ ID NO: 477 - DNA, 20 bp, Artificial Sequence
  source: /note="Description of Artificial Sequence: Synthetic oligonucleotide"
ccatccaagtcacttgggag

SEQ ID NO: 478 - DNA, 20 bp, Artificial Sequence
  source: /note="Description of Artificial Sequence: Synthetic oligonucleotide"
atgagatgcctggctgccat

SEQ ID NO: 479 - DNA, 20 bp, Artificial Sequence
  source: /note="Description of Artificial Sequence: Synthetic oligonucleotide"
ccatccaagtcacttgggag

SEQ ID NO: 480 - DNA, 20 bp, Artificial Sequence
  source: /note="Description of Artificial Sequence: Synthetic oligonucleotide"
atgagatgcctggctgccat

SEQ ID NO: 481 - DNA, 20 bp, Artificial Sequence
  source: /note="Description of Artificial Sequence: Synthetic oligonucleotide"
ccatccaagtcacttgggag

SEQ ID NO: 482 - DNA, 20 bp, Artificial Sequence
  source: /note="Description of Artificial Sequence: Synthetic oligonucleotide"
atgagatgcctggctgccat

SEQ ID NO: 483 - DNA, 20 bp, Artificial Sequence
  source: /note="Description of Artificial Sequence: Synthetic oligonucleotide"
ccatccaagtcacttgggag

SEQ ID NO: 484 - DNA, 20 bp, Artificial Sequence
  source: /note="Description of Artificial Sequence: Synthetic oligonucleotide"
atgagatgcctggctgccat

SEQ ID NO: 485 - DNA, 20 bp, Artificial Sequence
  source: /note="Description of Artificial Sequence: Synthetic oligonucleotide"
ccatccaagtcacttgggag

SEQ ID NO: 486 - DNA, 20 bp, Artificial Sequence
  source: /note="Description of Artificial Sequence: Synthetic oligonucleotide"
atgagatgcctggctgccat

SEQ ID NO: 487 - DNA, 20 bp, Artificial Sequence
  source: /note="Description of Artificial Sequence: Synthetic oligonucleotide"
gaagctttggttgggcaaca

SEQ ID NO: 488 - DNA, 20 bp, Artificial Sequence
  source: /note="Description of Artificial Sequence: Synthetic oligonucleotide"
atgagatgcctggctgccat

SEQ ID NO: 489 - DNA, 20 bp, Artificial Sequence
  source: /note="Description of Artificial Sequence: Synthetic oligonucleotide"
ccatccaagtcacttgggag

SEQ ID NO: 490 - DNA, 20 bp, Artificial Sequence
  source: /note="Description of Artificial Sequence: Synthetic oligonucleotide"
atgagatgcctggctgccat

SEQ ID NO: 491 - DNA, 20 bp, Artificial Sequence
  source: /note="Description of Artificial Sequence: Synthetic oligonucleotide"
gaagctttggttgggcaaca

SEQ ID NO: 492 - DNA, 20 bp, Artificial Sequence
  source: /note="Description of Artificial Sequence: Synthetic oligonucleotide"
atgagatgcctggctgccat

SEQ ID NO: 493 - DNA, 20 bp, Artificial Sequence
  source: /note="Description of Artificial Sequence: Synthetic oligonucleotide"
ccatccaagtcacttgggag

SEQ ID NO: 494 - DNA, 20 bp, Artificial Sequence
  source: /note="Description of Artificial Sequence: Synthetic oligonucleotide"
ccatccaagtcacttgggag

SEQ ID NO: 495 - DNA, 20 bp, Artificial Sequence
  source: /note="Description of Artificial Sequence: Synthetic oligonucleotide"
atgagatgcctggctgccat

SEQ ID NO: 496 - DNA, 20 bp, Artificial Sequence
  source: /note="Description of Artificial Sequence: Synthetic oligonucleotide"
ccatccaagtcacttgggag

SEQ ID NO: 497 - DNA, 20 bp, Artificial Sequence
  source: /note="Description of Artificial Sequence: Synthetic oligonucleotide"
ccatccaagtcacttgggag

SEQ ID NO: 498 - DNA, 20 bp, Artificial Sequence
  source: /note="Description of Artificial Sequence: Synthetic oligonucleotide"
ccatccaagtcacttgggag

SEQ ID NO: 499 - DNA, 20 bp, Artificial Sequence
  source: /note="Description of Artificial Sequence: Synthetic oligonucleotide"
ccatccaagtcacttgggag

SEQ ID NO: 500 - DNA, 20 bp, Artificial Sequence
  source: /note="Description of Artificial Sequence: Synthetic oligonucleotide"
ccatccaagtcacttgggag

SEQ ID NO: 501 - DNA, 20 bp, Artificial Sequence
  source: /note="Description of Artificial Sequence: Synthetic oligonucleotide"
ccatccaagtcacttgggag

SEQ ID NO: 502 - DNA, 20 bp, Artificial Sequence
  source: /note="Description of Artificial Sequence: Synthetic oligonucleotide"
ccatccaagtcacttgggag

SEQ ID NO: 503 - DNA, 20 bp, Artificial Sequence
  source: /note="Description of Artificial Sequence: Synthetic oligonucleotide"
ccatccaagtcacttgggag

SEQ ID NO: 504 - DNA, 20 bp, Artificial Sequence
  source: /note="Description of Artificial Sequence: Synthetic oligonucleotide"
ccatccaagtcacttgggag

SEQ ID NO: 505 - DNA, 20 bp, Artificial Sequence
  source: /note="Description of Artificial Sequence: Synthetic oligonucleotide"
ccatccaagtcacttgggag

SEQ ID NO: 506 - DNA, 20 bp, Artificial Sequence
  source: /note="Description of Artificial Sequence: Synthetic oligonucleotide"
tgagatgcctggctgccata

SEQ ID NO: 507 - DNA, 20 bp, Artificial Sequence
  source: /note="Description of Artificial Sequence: Synthetic oligonucleotide"
tgagatgcctggctgccata

SEQ ID NO: 508 - DNA, 20 bp, Artificial Sequence
  source: /note="Description of Artificial Sequence: Synthetic oligonucleotide"
tgagatgcctggctgccata

SEQ ID NO: 509 - DNA, 20 bp, Artificial Sequence
  source: /note="Description of Artificial Sequence: Synthetic oligonucleotide"
tgagatgcctggctgccata

SEQ ID NO: 510 - RNA, 20 nt, Artificial Sequence
  source: /note="Description of Artificial Sequence: Synthetic oligonucleotide"
uauggcagccaggcaucuca

SEQ ID NO: 511 - DNA, 20 bp, Artificial Sequence
  source: /note="Description of Artificial Sequence: Synthetic oligonucleotide"
tagccattgcagctgctcac

SEQ ID NO: 512 - DNA, 20 bp, Artificial Sequence
  source: /note="Description of Artificial Sequence: Synthetic oligonucleotide"
tagccattgcagctgctcac

SEQ ID NO: 513 - DNA, 20 bp, Artificial Sequence
  source: /note="Description of Artificial Sequence: Synthetic oligonucleotide"
tagccattgcagctgctcac

SEQ ID NO: 514 - DNA, 20 bp, Artificial Sequence
  source: /note="Description of Artificial Sequence: Synthetic oligonucleotide"
tagccattgcagctgctcac

SEQ ID NO: 515 - RNA, 20 nt, Artificial Sequence
  source: /note="Description of Artificial Sequence: Synthetic oligonucleotide"
gugagcagcugcaauggcua

SEQ ID NO: 516 - DNA, 20 bp, Artificial Sequence
  source: /note="Description of Artificial Sequence: Synthetic oligonucleotide"
tagccattgcagctgctcac

SEQ ID NO: 517 - DNA, 20 bp, Artificial Sequence
  source: /note="Description of Artificial Sequence: Synthetic oligonucleotide"
tagccattgcagctgctcac

SEQ ID NO: 518 - DNA, 20 bp, Artificial Sequence
  source: /note="Description of Artificial Sequence: Synthetic oligonucleotide"
tagccattgcagctgctcac

SEQ ID NO: 519 - DNA, 20 bp, Artificial Sequence
  source: /note="Description of Artificial Sequence: Synthetic oligonucleotide"
tagccattgcagctgctcac

SEQ ID NO: 520 - DNA, 20 bp, Artificial Sequence
  source: /note="Description of Artificial Sequence: Synthetic oligonucleotide"
tagccattgcagctgctcac

SEQ ID NO: 521 - RNA, 20 nt, Artificial Sequence
  source: /note="Description of Artificial Sequence: Synthetic oligonucleotide"
gugagcagcugcaauggcua

SEQ ID NO: 522 - DNA, 20 bp, Artificial Sequence
  source: /note="Description of Artificial Sequence: Synthetic oligonucleotide"
tccagttccttcattctgca

SEQ ID NO: 523 - DNA, 20 bp, Artificial Sequence
  source: /note="Description of Artificial Sequence: Synthetic oligonucleotide"
tccagttccttcattctgca

SEQ ID NO: 524 - DNA, 20 bp, Artificial Sequence
  source: /note="Description of Artificial Sequence: Synthetic oligonucleotide"
tccagttccttcattctgca

SEQ ID NO: 525 - DNA, 20 bp, Artificial Sequence
  source: /note="Description of Artificial Sequence: Synthetic oligonucleotide"
tccagttccttcattctgca

SEQ ID NO: 526 - DNA, 20 bp, Artificial Sequence
  source: /note="Description of Artificial Sequence: Synthetic oligonucleotide"
tccagttccttcattctgca

SEQ ID NO: 527 - RNA, 20 nt, Artificial Sequence
  source: /note="Description of Artificial Sequence: Synthetic oligonucleotide"
ugcagaaugaaggaacugga

SEQ ID NO: 528 - DNA, 20 bp, Artificial Sequence
  source: /note="Description of Artificial Sequence: Synthetic oligonucleotide"
tgagatgcctggctgccata

SEQ ID NO: 529 - DNA, 20 bp, Artificial Sequence
  source: /note="Description of Artificial Sequence: Synthetic oligonucleotide"
tgagatgcctggctgccata

SEQ ID NO: 530 - DNA, 20 bp, Artificial Sequence
  source: /note="Description of Artificial Sequence: Synthetic oligonucleotide"
tgagatgcctggctgccata

SEQ ID NO: 531 - DNA, 20 bp, Artificial Sequence
  source: /note="Description of Artificial Sequence: Synthetic oligonucleotide"
tgagatgcctggctgccata

SEQ ID NO: 532 - DNA, 20 bp, Artificial Sequence
  source: /note="Description of Artificial Sequence: Synthetic oligonucleotide"
tgagatgcctggctgccata

SEQ ID NO: 533 - RNA, 20 nt, Artificial Sequence
  source: /note="Description of Artificial Sequence: Synthetic oligonucleotide"
uauggcagccaggcaucuca

SEQ ID NO: 534 - DNA, 20 bp, Artificial Sequence
  source: /note="Description of Artificial Sequence: Synthetic oligonucleotide"
gcctcagtctgcttcgcacc

SEQ ID NO: 535 - DNA, 27 bp, Artificial Sequence
  source: /note="Description of Artificial Sequence: Synthetic oligonucleotide"
gcgtttgctcttcttcttgcgtttttt

SEQ ID NO: 536 - DNA, 20 bp, Artificial Sequence
  source: /note="Description of Artificial Sequence: Synthetic oligonucleotide"
gtccctgaagatgtcaatgc

SEQ ID NO: 537 - DNA, 20 bp, Artificial Sequence
  source: /note="Description of Artificial Sequence: Synthetic oligonucleotide"
tccagttccttcattctgca

SEQ ID NO: 538 - DNA, 20 bp, Artificial Sequence
  source: /note="Description of Artificial Sequence: Synthetic oligonucleotide"
tgagatgcctggctgccata

SEQ ID NO: 539 - DNA, 20 bp, Artificial Sequence
  source: /note="Description of Artificial Sequence: Synthetic oligonucleotide"
tagccattgcagctgctcac

SEQ ID NO: 540 - DNA, 20 bp, Artificial Sequence
  source: /note="Description of Artificial Sequence: Synthetic oligonucleotide"
tccagttccttcattctgca

SEQ ID NO: 541 - DNA, 20 bp, Artificial Sequence
  source: /note="Description of Artificial Sequence: Synthetic oligonucleotide"
tgagatgcctggctgccata

SEQ ID NO: 542 - DNA, 20 bp, Artificial Sequence
  source: /note="Description of Artificial Sequence: Synthetic oligonucleotide"
tagccattgcagctgctcac

SEQ ID NO: 543 - DNA, 20 bp, Artificial Sequence
  source: /note="Description of Artificial Sequence: Synthetic oligonucleotide"
tccagttccttcattctgca

SEQ ID NO: 544 - DNA, 20 bp, Artificial Sequence
  source: /note="Description of Artificial Sequence: Synthetic oligonucleotide"
tgagatgcctggctgccata

SEQ ID NO: 545 - DNA, 20 bp, Artificial Sequence
  source: /note="Description of Artificial Sequence: Synthetic oligonucleotide"
tagccattgcagctgctcac

SEQ ID NO: 546 - DNA, 20 bp, Artificial Sequence
  source: /note="Description of Artificial Sequence: Synthetic oligonucleotide"
tccagttccttcattctgca

SEQ ID NO: 547 - DNA, 20 bp, Artificial Sequence
  source: /note="Description of Artificial Sequence: Synthetic oligonucleotide"
tgagatgcctggctgccata

SEQ ID NO: 548 - DNA, 20 bp, Artificial Sequence
  source: /note="Description of Artificial Sequence: Synthetic oligonucleotide"
tagccattgcagctgctcac

SEQ ID NO: 549 - DNA, 20 bp, Artificial Sequence
  source: /note="Description of Artificial Sequence: Synthetic oligonucleotide"
tccagttccttcattctgca

SEQ ID NO: 550 - DNA, 20 bp, Artificial Sequence
  source: /note="Description of Artificial Sequence: Synthetic oligonucleotide"
tgagatgcctggctgccata

SEQ ID NO: 551 - DNA, 20 bp, Artificial Sequence
  source: /note="Description of Artificial Sequence: Synthetic oligonucleotide"
tagccattgcagctgctcac

SEQ ID NO: 552 - DNA, 20 bp, Artificial Sequence
  source: /note="Description of Artificial Sequence: Synthetic oligonucleotide"
  source: /note="Description of Combined DNA/RNA Molecule: Synthetic oligonucleotide"
uagccattgcagctgctcac

SEQ ID NO: 553 - DNA, 16 bp, Artificial Sequence
  source: /note="Description of Artificial Sequence: Synthetic oligonucleotide"
  source: /note="Description of Combined DNA/RNA Molecule: Synthetic oligonucleotide"
uagccattgcagctgc

SEQ ID NO: 554 - DNA, 20 bp, Artificial Sequence
  source: /note="Description of Artificial Sequence: Synthetic oligonucleotide"
tagccattgcagctgctcac

SEQ ID NO: 555 - DNA, 20 bp, Artificial Sequence
  source: /note="Description of Artificial Sequence: Synthetic oligonucleotide"
attaataaattgtcatcacc

SEQ ID NO: 556 - RNA, 20 nt, Artificial Sequence
  source: /note="Description of Artificial Sequence: Synthetic oligonucleotide"
ggugcgaagcagacugaggc

SEQ ID NO: 557 - RNA, 20 nt, Artificial Sequence
  source: /note="Description of Artificial Sequence: Synthetic oligonucleotide"
ugcagaaugaaggaacugga

SEQ ID NO: 558 - RNA, 20 nt, Artificial Sequence
  source: /note="Description of Artificial Sequence: Synthetic oligonucleotide"
uauggcagccaggcaucuca

SEQ ID NO: 559 - RNA, 20 nt, Artificial Sequence
  source: /note="Description of Artificial Sequence: Synthetic oligonucleotide"
gugagcagcugcaauggcua

SEQ ID NO: 560 - DNA, 20 bp, Artificial Sequence
  source: /note="Description of Artificial Sequence: Synthetic oligonucleotide"
tagccattgcagctgctcac

SEQ ID NO: 561 - RNA, 20 nt, Artificial Sequence
  source: /note="Description of Artificial Sequence: Synthetic oligonucleotide"
gugagcggcugcaauggcua

SEQ ID NO: 562 - RNA, 20 nt, Artificial Sequence
  source: /note="Description of Artificial Sequence: Synthetic oligonucleotide"
gugagcagcugcgauggcua

SEQ ID NO: 563 - RNA, 20 nt, Artificial Sequence
  source: /note="Description of Artificial Sequence: Synthetic oligonucleotide"
ggugaugacaauuuauuaau

SEQ ID NO: 564 - RNA, 20 nt, Artificial Sequence
  source: /note="Description of Artificial Sequence: Synthetic oligonucleotide"
ggugauggcaauuuauuaau

SEQ ID NO: 565 - DNA, 20 bp, Artificial Sequence
  source: /note="Description of Artificial Sequence: Synthetic oligonucleotide"
tgagatgcctggctgccata

SEQ ID NO: 566 - DNA, 20 bp, Artificial Sequence
  source: /note="Description of Artificial Sequence: Synthetic oligonucleotide"
tgagatgcctggctgccata

SEQ ID NO: 567 - DNA, 20 bp, Artificial Sequence
  source: /note="Description of Artificial Sequence: Synthetic oligonucleotide"
tgagatgcctggctgccata

SEQ ID NO: 568 - DNA, 20 bp, Artificial Sequence
  source: /note="Description of Artificial Sequence: Synthetic oligonucleotide"
tagccattgcagctgctcac

SEQ ID NO: 569 - DNA, 20 bp, Artificial Sequence
  source: /note="Description of Artificial Sequence: Synthetic oligonucleotide"
tagccattgcagctgctcac

SEQ ID NO: 570 - DNA, 20 bp, Artificial Sequence
  source: /note="Description of Artificial Sequence: Synthetic oligonucleotide"
tagccattgcagctgctcac

SEQ ID NO: 571 - DNA, 20 bp, Artificial Sequence
  source: /note="Description of Artificial Sequence: Synthetic oligonucleotide"
tagccattgcagctgctcac

SEQ ID NO: 572 - DNA, 20 bp, Artificial Sequence
  source: /note="Description of Artificial Sequence: Synthetic oligonucleotide"
tagccattgcagctgctcac

SEQ ID NO: 573 - DNA, 20 bp, Artificial Sequence
  source: /note="Description of Artificial Sequence: Synthetic oligonucleotide"
tagccattgcagctgctcac

SEQ ID NO: 574 - DNA, 20 bp, Artificial Sequence
  source: /note="Description of Artificial Sequence: Synthetic oligonucleotide"
tagccattgcagctgctcac

SEQ ID NO: 575 - DNA, 20 bp, Artificial Sequence
  source: /note="Description of Artificial Sequence: Synthetic oligonucleotide"
tagccattgcagctgctcac

SEQ ID NO: 576 - DNA, 20 bp, Artificial Sequence
  source: /note="Description of Artificial Sequence: Synthetic oligonucleotide"
tagccattgcagctgctcac

SEQ ID NO: 577 - DNA, 20 bp, Artificial Sequence
  source: /note="Description of Artificial Sequence: Synthetic oligonucleotide"
tagccattgcagctgctcac

SEQ ID NO: 578 - DNA, 20 bp, Artificial Sequence
  source: /note="Description of Artificial Sequence: Synthetic oligonucleotide"
tagccattgcagctgctcac

SEQ ID NO: 579 - DNA, 20 bp, Artificial Sequence
  source: /note="Description of Artificial Sequence: Synthetic oligonucleotide"
tagccattgcagctgctcac

SEQ ID NO: 580 - DNA, 20 bp, Artificial Sequence
  source: /note="Description of Artificial Sequence: Synthetic oligonucleotide"
tagccattgcagctgctcac

SEQ ID NO: 581 - DNA, 20 bp, Artificial Sequence
  source: /note="Description of Artificial Sequence: Synthetic oligonucleotide"
tagccattgcagctgctcac

SEQ ID NO: 582 - DNA, 20 bp, Artificial Sequence
  source: /note="Description of Artificial Sequence: Synthetic oligonucleotide"
tagccattgcagctgctcac

SEQ ID NO: 583 - DNA, 20 bp, Artificial Sequence
  source: /note="Description of Artificial Sequence: Synthetic oligonucleotide"
tagccattgcagctgctcac

SEQ ID NO: 584 - DNA, 20 bp, Artificial Sequence
  source: /note="Description of Artificial Sequence: Synthetic oligonucleotide"
tagccattgcagctgctcac

SEQ ID NO: 585 - DNA, 20 bp, Artificial Sequence
  source: /note="Description of Artificial Sequence: Synthetic oligonucleotide"
tagccattgcagctgctcac

SEQ ID NO: 586 - DNA, 20 bp, Artificial Sequence
  source: /note="Description of Artificial Sequence: Synthetic oligonucleotide"
tagccattgcagctgctcac

SEQ ID NO: 587 - DNA, 20 bp, Artificial Sequence
  source: /note="Description of Artificial Sequence: Synthetic oligonucleotide"
tagccattgcagctgctcac

SEQ ID NO: 588 - DNA, 20 bp, Artificial Sequence
  source: /note="Description of Artificial Sequence: Synthetic oligonucleotide"
tagccattgcagctgctcac

SEQ ID NO: 589 - DNA, 20 bp, Artificial Sequence
  source: /note="Description of Artificial Sequence: Synthetic oligonucleotide"
tagccattgcagctgctcac

SEQ ID NO: 590 - DNA, 20 bp, Artificial Sequence
  source: /note="Description of Artificial Sequence: Synthetic oligonucleotide"
tagccattgcagctgctcac

SEQ ID NO: 591 - DNA, 20 bp, Artificial Sequence
  source: /note="Description of Artificial Sequence: Synthetic oligonucleotide"
tagccattgcagctgctcac

SEQ ID NO: 592 - DNA, 20 bp, Artificial Sequence
  source: /note="Description of Artificial Sequence: Synthetic oligonucleotide"
tagccattgcagctgctcac

SEQ ID NO: 593 - DNA, 20 bp, Artificial Sequence
  source: /note="Description of Artificial Sequence: Synthetic oligonucleotide"
attaataaattgtcatcacc

SEQ ID NO: 594 - DNA, 20 bp, Artificial Sequence
  source: /note="Description of Artificial Sequence: Synthetic oligonucleotide"
attaataaattgtcatcacc

SEQ ID NO: 595 - DNA, 20 bp, Artificial Sequence
  source: /note="Description of Artificial Sequence: Synthetic oligonucleotide"
gcctcagtctgcttcgcacc

SEQ ID NO: 596 - DNA, 20 bp, Artificial Sequence
  source: /note="Description of Artificial Sequence: Synthetic oligonucleotide"
gcctcagtctgcttcgcacc

SEQ ID NO: 597 - DNA, 20 bp, Artificial Sequence
  source: /note="Description of Artificial Sequence: Synthetic oligonucleotide"
gcctcagtctgcttcgcacc

SEQ ID NO: 598 - DNA, 20 bp, Artificial Sequence
  source: /note="Description of Artificial Sequence: Synthetic oligonucleotide"
gcctcagtctgcttcgcacc

SEQ ID NO: 599 - DNA, 20 bp, Artificial Sequence
  source: /note="Description of Artificial Sequence: Synthetic oligonucleotide"
gcctcagtctgcttcgcacc

SEQ ID NO: 600 - DNA, 20 bp, Artificial Sequence
  source: /note="Description of Artificial Sequence: Synthetic oligonucleotide"
gtccctgaagatgtcaatgc

SEQ ID NO: 601 - DNA, 20 bp, Artificial Sequence
  source: /note="Description of Artificial Sequence: Synthetic oligonucleotide"
gtccctgaagatgtcaatgc

SEQ ID NO: 602 - DNA, 20 bp, Artificial Sequence
  source: /note="Description of Artificial Sequence: Synthetic oligonucleotide"
gtccctgaagatgtcaatgc

SEQ ID NO: 603 - DNA, 20 bp, Artificial Sequence
  source: /note="Description of Artificial Sequence: Synthetic oligonucleotide"
gtccctgaagatgtcaatgc

SEQ ID NO: 604 - DNA, 20 bp, Artificial Sequence
  source: /note="Description of Artificial Sequence: Synthetic oligonucleotide"
gcctcagtctgcttcgcacc

SEQ ID NO: 605 - DNA, 20 bp, Artificial Sequence
  source: /note="Description of Artificial Sequence: Synthetic oligonucleotide"
gcctcagtctgcttcgcacc

SEQ ID NO: 606 - DNA, 20 bp, Artificial Sequence
  source: /note="Description of Artificial Sequence: Synthetic oligonucleotide"
gcctcagtctgcttcgcacc

SEQ ID NO: 607 - DNA, 20 bp, Artificial Sequence
  source: /note="Description of Artificial Sequence: Synthetic oligonucleotide"
gcctcagtctgcttcgcacc

SEQ ID NO: 608 - DNA, 20 bp, Artificial Sequence
  source: /note="Description of Artificial Sequence: Synthetic oligonucleotide"
gcctcagtctgcttcgcacc

SEQ ID NO: 609 - DNA, 20 bp, Artificial Sequence
  source: /note="Description of Artificial Sequence: Synthetic oligonucleotide"
gcctcagtctgcttcgcacc

SEQ ID NO: 610 - DNA, 20 bp, Artificial Sequence
  source: /note="Description of Artificial Sequence: Synthetic oligonucleotide"
  source: /note="Description of Combined DNA/RNA Molecule: Synthetic oligonucleotide"
uagccattgcagctgctcac

SEQ ID NO: 611 - DNA, 20 bp, Artificial Sequence
  source: /note="Description of Artificial Sequence: Synthetic oligonucleotide"
  source: /note="Description of Combined DNA/RNA Molecule: Synthetic oligonucleotide"
uagccattgcagctgctcac

SEQ ID NO: 612 - DNA, 16 bp, Artificial Sequence
  source: /note="Description of Artificial Sequence: Synthetic oligonucleotide"
  source: /note="Description of Combined DNA/RNA Molecule: Synthetic oligonucleotide"
uagccattgcagctgc

SEQ ID NO: 613 - DNA, 20 bp, Artificial Sequence
  source: /note="Description of Artificial Sequence: Synthetic oligonucleotide"
tagccattgcagctgctcac

SEQ ID NO: 614 - DNA, 20 bp, Artificial Sequence
  source: /note="Description of Artificial Sequence: Synthetic oligonucleotide"
tagccattgcagctgctcac

SEQ ID NO: 615 - DNA, 20 bp, Artificial Sequence
  source: /note="Description of Artificial Sequence: Synthetic oligonucleotide"
tagccattgcagctgctcac

SEQ ID NO: 616 - DNA, 20 bp, Artificial Sequence
  source: /note="Description of Artificial Sequence: Synthetic oligonucleotide"
tagccattgcagctgctcac

SEQ ID NO: 617 - DNA, 20 bp, Artificial Sequence
  source: /note="Description of Artificial Sequence: Synthetic oligonucleotide"
tagccattgcagctgctcac

SEQ ID NO: 618 - DNA, 20 bp, Artificial Sequence
  source: /note="Description of Artificial Sequence: Synthetic oligonucleotide"
tagccattgcagctgctcac

SEQ ID NO: 619 - DNA, 20 bp, Artificial Sequence
  source: /note="Description of Artificial Sequence: Synthetic oligonucleotide"
tagccattgcagctgctcac

SEQ ID NO: 620 - DNA, 20 bp, Artificial Sequence
  source: /note="Description of Artificial Sequence: Synthetic oligonucleotide"
tagccattgcagctgctcac

SEQ ID NO: 621 - protein, 6 aa, Artificial Sequence
  source: /note="Description of Artificial Sequence: Synthetic 6xHis tag"
HHHHHH